European Patent Specification EP 3 849 595 B1, published November 19, 2025. Title: POLYNUCLEOTIDES ENCODING GLUCOSE-6-PHOSPHATASE FOR THE TREATMENT OF GLYCOGEN STORAGE DISEASE. Applicant: MODERNATX, INC. The sequence listing filed with the application follows.

SEQUENCE LISTING (235 sequences)

SEQ ID NO: 1 - protein, 365 aa, Artificial Sequence
  source: /note="Description of Artificial Sequence: Synthetic polypeptide"
MEEGMNVLHDFGIQSTHYLQVNYQDSQDWFILVSVIADLRNAFYVLFPIWFHLQEAVGIKLLWVAVIGDWLNLVFKWILFGQRPYWWVLDTDYYSNTSVPLIKQFPVTCETGPGSPSGHAMGTAGVYYVMVTSTLSIFQGKIKPTYRFRCLNVILWLGFWAVQLNVCLSRIYLAAHFPHQVVAGVLSGIAVAETFSHIHSIYNASLKKYFLITFFLFSFAIGFYLLLKGLGVDLLWTLEKAQRWCEQPEWVHIDTTPFASLLKNLGTLFGLGLALNSSMYRESCKGKLSKWLPFRLSSIVASLVLLHVFDSLKPPSQVELVFYVLSFCKSAVVPLASVSVIPYCLAQVLGQPHKKSLDYKDDDDK

SEQ ID NO: 2 - RNA, 1095 nt, Artificial Sequence
  source: /note="Description of Artificial Sequence: Synthetic polynucleotide"
auggaggaaggaaugaauguucuccaugacuuugggauccagucaacacauuaccuccaggugaauuaccaagacucccaggacugguucaucuugguguccgugaucgcagaccucaggaaugccuucuacguccucuuccccaucugguuccaucuucaggaagcugugggcauuaaacuccuuuggguagcugugauuggagacuggcucaaccucgucuuuaaguggauucucuuuggacagcguccauacugguggguuuuggauacugacuacuacagcaacacuuccgugccccugauaaagcaguucccuguaaccugugagacuggaccagggagccccucuggccaugccaugggcacagcagguguauacuacgugauggucacaucuacucuuuccaucuuucagggaaagauaaagccgaccuacagauuucggugcuugaaugucauuuugugguugggauucugggcugugcagcugaaugucugucugucacgaaucuaccuugcugcucauuuuccucaucaaguuguugcuggaguccugucaggcauugcuguugcagaaacuuucagccacauccacagcaucuauaaugccagccucaagaaauauuuucucauuaccuucuuccuguucagcuucgccaucggauuuuaucugcugcucaagggacuggguguagaccuccuguggacucuggagaaagcccagagguggugcgagcagccagaauggguccacauugacaccacacccuuugccagccuccucaagaaccugggcacgcucuuuggccuggggcuggcucucaacuccagcauguacagggagagcugcaaggggaaacucagcaaguggcucccauuccgccucagcucuauuguagccucccucguccuccugcacgucuuugacuccuugaaacccccaucccaagucgagcuggucuucuacgucuuguccuucugcaagagugcgguagugccccuggcauccgucagugucauccccuacugccucgcccagguccugggccagccgcacaagaagucguuggacuacaaggacgacgaugacaag

SEQ ID NO: 3 - RNA, 47 nt, Artificial Sequence
  source: /note="Description of Artificial Sequence: Synthetic oligonucleotide"
gggaaauaagagagaaaagaagaguaagaagaaauauaagagccacc

SEQ ID NO: 4 - RNA, 142 nt, Artificial Sequence
  source: /note="Description of Artificial Sequence: Synthetic polynucleotide"
ugauaauaggcuggagccucgguggccuagcuucuugccccuugggccuccccccagccccuccuccccuuccugcacccguacccccuccauaaaguaggaaacacuacaguggucuuugaauaaagucugagugggcggc

SEQ ID NO: 5 - RNA, 1071 nt, Artificial Sequence
  source: /note="Description of Artificial Sequence: Synthetic polynucleotide"
auggaggaaggaaugaacauucuccaugacuuugggauccagucgacucgcuaucuccaagugaauuaccaagacucccaggacugguucauccuugugucugugauugcugaccugaggaacgccuucuauguccucuuucccaucugguuccaucuuaaagagacugugggcaucaaucuccucuggguggcaguggucggagacugguucaaccucgucuucaaguggauucuguuuggacaacgcccguauugguggguccuggacaccgacuacuacagcaacagcuccgugccuauaauaaagcaguucccugucaccugugagaccggaccaggaagucccucuggccaugccaugggcgcagcagguguauacuauguuauggucacuucuacucuugcuaucuuucgaggaaagaaaaagccaacguauggauuccgguguuugaacgucaucuugugguugggauucugggcugugcagcugaacgucugucugucccggaucuaccuugcugcucacuuuccccaccaggucguggcuggagucuugucaggcauugcuguggcugaaacuuucagccacauccggggcaucuacaaugccagccuccggaaguauugucucaucaccaucuucuuguuugguuucgcgcuuggauucuaccugcuacuaaaagggcuagggguggaccuccuguggacuuuggagaaagcuaagagauggugugagcggccagaauggguccaccuugacacuacacccuuugccagccucuucaaaaaccugggaacccucuugggguuggggcuggcccucaacuccagcauguaccggaagagcugcaagggagaacucagcaaguugcucccauuccgcuucgccugcauuguggcuuccuugguccuccugcaucucuuugacucucugaagcccccaucccagguugaguugaucuucuacaucuugucuuucugcaagagcgcaacaguucccuuugcaucugucagucuuaucccauacugccuagcccggauccugggacagacacacaagaagucuuug

SEQ ID NO: 6 - RNA, 1095 nt, Artificial Sequence
  source: /note="Description of Artificial Sequence: Synthetic polynucleotide"
auggaggaaggaaugaacauucuccaugacuuugggauccagucgacucgcuaucuccaagugaauuaccaagacucccaggacugguucauccuugugucugugauugcugaccugaggaacgccuucuauguccucuuucccaucugguuccaucuuaaagagacugugggcaucaaucuccucuggguggcaguggucggagacugguucaaccucgucuucaaguggauucuguuuggacaacgcccguauugguggguccuggacaccgacuacuacagcaacagcuccgugccuauaauaaagcaguucccugucaccugugagaccggaccaggaagucccucuggccaugccaugggcgcagcagguguauacuauguuauggucacuucuacucuugcuaucuuucgaggaaagaaaaagccaacguauggauuccgguguuugaacgucaucuugugguugggauucugggcugugcagcugaacgucugucugucccggaucuaccuugcugcucacuuuccccaccaggucguggcuggagucuugucaggcauugcuguggcugaaacuuucagccacauccggggcaucuacaaugccagccuccggaaguauugucucaucaccaucuucuuguuugguuucgcgcuuggauucuaccugcuacuaaaagggcuagggguggaccuccuguggacuuuggagaaagcuaagagauggugugagcggccagaauggguccaccuugacacuacacccuuugccagccucuucaaaaaccugggaacccucuugggguuggggcuggcccucaacuccagcauguaccggaagagcugcaagggagaacucagcaaguugcucccauuccgcuucgccugcauuguggcuuccuugguccuccugcaucucuuugacucucugaagcccccaucccagguugaguugaucuucuacaucuugucuuucugcaagagcgcaacaguucccuuugcaucugucagucuuaucccauacugccuagcccggauccugggacagacacacaagaagucuuuggacuacaaggacgacgaugacaag

SEQ ID NO: 7 - RNA, 1071 nt, Artificial Sequence
  source: /note="Description of Artificial Sequence: Synthetic polynucleotide"
auggaggaaggaaugaauguucuccaugacuuugggauccagucaacacauuaccuccaggugaauuaccaagacucccaggacugguucaucuugguguccgugaucgcagaccucaggaaugccuucuacguccucuuccccaucugguuccaucuucaggaagcugugggcauuaaacuccuuuggguagcugugauuggagacuggcucaaccucgucuuuaaguggauucucuuuggacagcguccauacugguggguuuuggauacugacuacuacagcaacacuuccgugccccugauaaagcaguucccuguaaccugugagacuggaccagggagccccucuggccaugccaugggcacagcagguguauacuacgugauggucacaucuacucuuuccaucuuucagggaaagauaaagccgaccuacagauuucggugcuugaaugucauuuugugguugggauucugggcugugcagcugaaugucugucugucacgaaucuaccuugcugcucauuuuccucaucaaguuguugcuggaguccugucaggcauugcuguugcagaaacuuucagccacauccacagcaucuauaaugccagccucaagaaauauuuucucauuaccuucuuccuguucagcuucgccaucggauuuuaucugcugcucaagggacuggguguagaccuccuguggacucuggagaaagcccagagguggugcgagcagccagaauggguccacauugacaccacacccuuugccagccuccucaagaaccugggcacgcucuuuggccuggggcuggcucucaacuccagcauguacagggagagcugcaaggggaaacucagcaaguggcucccauuccgccucagcucuauuguagccucccucguccuccugcacgucuuugacuccuugaaacccccaucccaagucgagcuggucuucuacgucuuguccuucugcaagagugcgguagugccccuggcauccgucagugucauccccuacugccucgcccagguccugggccagccgcacaagaagucguug

SEQ ID NO: 8 - RNA, 1071 nt, Artificial Sequence
  source: /note="Description of Artificial Sequence: Synthetic polynucleotide"
auggaggaaggaaugaauguucuccaugacuuugggauccagucaacacauuaccuccaggugaauuaccaagacucccaggacugguucaucuugguguccgugaucgcagaccucaggaaugccuucuacguccucuuccccaucugguuccaucuucaggaagcugugggcauuaaacuccuuuggguagcugugauuggagacuggcucaaccucgucuuuaaguggauucucuuuggacagcguccauacugguggguuuuggauacugacuacuacagcaacacuuccgugccccugauaaagcaguucccuguaaccugugagacuggaccagggagccccucuggccaugccaugggcacagcagguguauacuacgugauggucacaucuacucuuuccaucuuuaggggaaagauaaagccgaccuacagauuucggugcuugaaugucauuuugugguugggauucugggcugugcagcugaaugucugucugucacgaaucuaccuugcugcucauuuuccucaucaaguuguugcuggaguccugucaggcauugcuguugcagaaacuuucagccacauccacagcaucuauaaugccagccucaagaaauauuuucucauuaccuucuuccuguucagcuucgccaucggauuuuaucugcugcucaagggacuggguguagaccuccuguggacucuggagaaagcccagagguggugcgagaggccagaauggguccacauugacaccacacccuuugccagccuccucaagaaccugggcacgcucuuuggccuggggcuggcucucaacuccagcauguacagggagagcugcaaggggaaacucagcaaguggcucccauuccgccucagcuguauuguagccucccucguccuccugcacgucuuugacuccuugaaacccccaucccaagucgagcuggucuucuacgucuuguccuucugcaagagugcgguagugccccuggcauccgucagugucauccccuacugccucgcccagguccugggccagccgcacaagaagucguug

SEQ ID NO: 9 - RNA, 1071 nt, Artificial Sequence
  source: /note="Description of Artificial Sequence: Synthetic polynucleotide"
auggaggaaggaaugaauguucuccaugacuuugggauccagucaacacauuaccuccaggugaauuaccaagacucccaggacugguucaucuugguguccgugaucgcagaccucaggaaugccuucuacguccucuuccccaucugguuccaucuucaggaagcugugggcauuaaacuccuuuggguagcugugauuggagacuggcucaaccucgucuuuaaguggauucucuuuggacagcguccauacugguggguuuuggauacugacuacuacagcaacacuuccgugccccugauaaagcaguucccuguaaccugugagacuggaccagggagccccucuggccaugccaugggcacagcagguguauacuacgugauggucacaucuacucuuuccaucuuucagggaaagauaaagccgaccuacagauuucggugcuugaaugucauuuugugguugggauucugggcugugcagcugaaugucugucugucacgaaucuaccuugcugcucauuuuccucaucaaguuguugcuggaguccugucaggcauugcuguugcagaaacuuucagccacauccacagcaucuauaaugccagccucaagaaauauuuucucauuaccuucuuccuguucagcuucgccaucggauuuuaucugcugcucaagggacuggguguagaccuccuguggacucuggagaaagcccagagguggugcgagcagccagaauggguccacauugacaccacacccuuugccagccuccucaagaaccugggcacgcucuuuggccuggggcuggcucucaacuccagcauguacagggagagcugcaaggggaaacucagcaaguggcucccauuccgccucggcuguauuguagccucccucguccuccugcaccucuuugacuccuugaaacccccaucccaagucgagcugaucuucuacgucuuguccuucugcaagagugcgguagugccccuggcauccgucagucucauccccuacugccucgcccagguccugggccagccgcacaagaagucguug

SEQ ID NO: 10 - RNA, 1071 nt, Artificial Sequence
  source: /note="Description of Artificial Sequence: Synthetic polynucleotide"
auggaggaaggaaugaauguucuccaugacuuugggauccagucaacacauuaccuccaggugaauuaccaagacucccaggacugguucaucuugguguccgugaucgcagaccucaggaaugccuucuacguccucuuccccaucugguuccaucuucaggaagcugugggcauuaaacuccuuuggguagcugugauuggagacuggcucaaccucgucuuuaaguggauucucuuuggacagcguccauacugguggguuuuggauacugacuacuacagcaacacuuccgugccccugauaaagcaguucccuguaaccugugagacuggaccagggagccccucuggccaugccaugggcacagcagguguauacuacgugauggucacaucuacucuuuccaucuuuaggggaaagaagaagccgaccuacagauuucggugcuugaaugucauuuugugguugggauucugggcugugcagcugaaugucugucugucacgaaucuaccuugcugcucauuuuccucaucaaguuguugcuggaguccugucaggcauugcuguugcagaaacuuucagccacauccacagcaucuauaaugccagccucaagaaauauuuucucauuaccuucuuccuguucagcuucgccaucggauuuuaucugcugcucaagggacuggguguagaccuccuguggacucuggagaaagcccagagguggugcgagaggccagaauggguccacauugacaccacacccuuugccagccuccucaagaaccugggcacgcucuuuggccuggggcuggcucucaacuccagcauguacagggagagcugcaaggggaaacucagcaaguggcucccauuccgccucagcuguauuguagccucccucguccuccugcaccucuuugacuccuugaaacccccaucccaagucgagcuggucuucuacgucuuguccuucugcaagagugcgguagugccccuggcauccgucagugucauccccuacugccucgcccagguccugggccagccgcacaagaagucguug

SEQ ID NO: 11 - RNA, 1071 nt, Artificial Sequence
  source: /note="Description of Artificial Sequence: Synthetic polynucleotide"
auggaggaaggaaugaauguucuccaugacuuugggauccagucaacacauuaccuccaggugaauuaccaagacucccaggacugguucaucuugguguccgugaucgcagaccucaggaaugccuucuacguccucuuccccaucugguuccaucuucaggaagcugugggcauuaaacuccuuuggguagcugugauuggagacuggcucaaccucgucuuuaaguggauucucuuuggacagcguccauacugguggguuuuggauacugacuacuacagcaacacuuccgugccccugauaaagcaguucccuguaaccugugagacuggaccagggagccccucuggccaugccaugggcacagcagguguauacuacgugauggucacaucuacucuuuccaucuuucagggaaagauaaagccgaccuacagauuucggugcuugaaugucauuuugugguugggauucugggcugugcagcugaaugucugucugucacgaaucuaccuugcugcucauuuuccucaucaaguuguugcuggaguccugucaggcauugcuguugcagaaacuuucagccacauccacagcaucuauaaugccagccucaagaaauauuuucucauuaccuucuuccuguucagcuucgccaucggauuuuaucugcugcucaagggacuggguguagaccuccuguggacucuggagaaagcccagagguggugcgagcagccagaauggguccacauugacaccacacccuuugccagccuccucaagaaccugggcacgcucuuuggccuggggcuggcucucaacuccagcauguacagggagagcugcaaggggaaacucagcaaguggcucccauuccgccucagcucuauuguagccucccucguccuccugcacgucuuugacuccuugaaacccccaucccaagucgagcuggucuucuacgucuuguccuucugcaagagugcggcagugccccuggcauccgucagugucauccccuacugccucgcccagguccugggccagccgcacaagaagucguug

SEQ ID NO: 12 - RNA, 1071 nt, Artificial Sequence
  source: /note="Description of Artificial Sequence: Synthetic polynucleotide"
auggaggaaggaaugaauguucuccaugacuuugggauccagucaacacauuaccuccaggugaauuaccaagacucccaggacugguucaucuugguguccgugaucgcagaccucaggaaugccuucuacguccucuuccccaucugguuccaucuucaggaagcugugggcauuaaacuccuuuggguagcugugauuggagacuggcucaaccucgucuuuaaguggauucucuuuggacagcguccauacugguggguuuuggauacugacuacuacagcaacacuuccgugccccugauaaagcaguucccuguaaccugugagacuggaccagggagccccucuggccaugccaugggcacagcagguguauacuacgugauggucacaucuacucuuuccaucuuuaggggaaagauaaagccgaccuacagauuucggugcuugaaugucauuuugugguugggauucugggcugugcagcugaaugucugucugucacgaaucuaccuugcugcucauuuuccucaucaaguuguugcuggaguccugucaggcauugcuguugcagaaacuuucagccacauccacagcaucuauaaugccagccucaagaaauauuuucucauuaccuucuuccuguucagcuucgccaucggauuuuaucugcugcucaagggacuggguguagaccuccuguggacucuggagaaagcccagagguggugcgagcagccagaauggguccacauugacaccacacccuuugccagccuccucaagaaccugggcacgcucuuuggccuggggcuggcucucaacuccagcauguacagggagagcugcaaggggaaacucagcaaguggcucccauuccgccucagcucuauuguagccucccucguccuccugcacgucuuugacuccuugaaacccccaucccaagucgagcuggucuucuacgucuuguccuucugcaagagugcgguagugccccuggcauccgucagugucauccccuacugccucgcccagguccugggccagccgcacaagaagucguug

SEQ ID NO: 13 - RNA, 1071 nt, Artificial Sequence
  source: /note="Description of Artificial Sequence: Synthetic polynucleotide"
auggaggaaggaaugaauguucuccaugacuuugggauccagucaacacauuaccuccaggugaauuaccaagacucccaggacugguucaucuugguguccgugaucgcagaccucaggaaugccuucuacguccucuuccccaucugguuccaucuucaggaagcugugggcauuaaacuccuuuggguagcugugauuggagacuggcucaaccucgucuuuaaguggauucucuuuggacagcguccauacugguggguuuuggauacugacuacuacagcaacacuuccgugccccugauaaagcaguucccuguaaccugugagacuggaccagggagccccucuggccaugccaugggcacagcagguguauacuacgugauggucacaucuacucuuuccaucuuucagggaaagaagaagccgaccuacagauuucggugcuugaaugucauuuugugguugggauucugggcugugcagcugaaugucugucugucacgaaucuaccuugcugcucauuuuccucaucaaguuguugcuggaguccugucaggcauugcuguugcagaaacuuucagccacauccacagcaucuauaaugccagccucaagaaauauuuucucauuaccuucuuccuguucagcuucgccaucggauuuuaucugcugcucaagggacuggguguagaccuccuguggacucuggagaaagcccagagguggugcgagcagccagaauggguccacauugacaccacacccuuugccagccuccucaagaaccugggcacgcucuuuggccuggggcuggcucucaacuccagcauguacagggagagcugcaaggggaaacucagcaaguggcucccauuccgccucagcucuauuguagccucccucguccuccugcacgucuuugacuccuugaaacccccaucccaagucgagcuggucuucuacgucuuguccuucugcaagagugcgguagugccccuggcauccgucagugucauccccuacugccucgcccagguccugggccagccgcacaagaagucguug

SEQ ID NO: 14 - RNA, 1071 nt, Artificial Sequence
  source: /note="Description of Artificial Sequence: Synthetic polynucleotide"
auggaggaaggaaugaauguucuccaugacuuugggauccagucaacacauuaccuccaggugaauuaccaagacucccaggacugguucaucuugguguccgugaucgcagaccucaggaaugccuucuacguccucuuccccaucugguuccaucuucaggaagcugugggcauuaaacuccuuuggguagcugugauuggagacuggcucaaccucgucuuuaaguggauucucuuuggacagcguccauacugguggguuuuggauacugacuacuacagcaacacuuccgugccccugauaaagcaguucccuguaaccugugagacuggaccagggagccccucuggccaugccaugggcacagcagguguauacuacgugauggucacaucuacucuuuccaucuuucagggaaagauaaagccgaccuacagauuucggugcuugaaugucauuuugugguugggauucugggcugugcagcugaaugucugucugucacgaaucuaccuugcugcucauuuuccucaucaaguuguugcuggaguccugucaggcauugcuguugcagaaacuuucagccacauccacagcaucuauaaugccagccucaagaaauauuuucucauuaccuucuuccuguucagcuucgccaucggauuuuaucugcugcucaagggacuggguguagaccuccuguggacucuggagaaagcccagagguggugcgagaggccagaauggguccacauugacaccacacccuuugccagccuccucaagaaccugggcacgcucuuuggccuggggcuggcucucaacuccagcauguacagggagagcugcaaggggaaacucagcaaguggcucccauuccgccucagcucuauuguagccucccucguccuccugcacgucuuugacuccuugaaacccccaucccaagucgagcuggucuucuacgucuuguccuucugcaagagugcgguagugccccuggcauccgucagugucauccccuacugccucgcccagguccugggccagccgcacaagaagucguug

SEQ ID NO: 15 - RNA, 1071 nt, Artificial Sequence
  source: /note="Description of Artificial Sequence: Synthetic polynucleotide"
auggaggaaggaaugaauguucuccaugacuuugggauccagucaacacauuaccuccaggugaauuaccaagacucccaggacugguucaucuugguguccgugaucgcagaccucaggaaugccuucuacguccucuuccccaucugguuccaucuucaggaagcugugggcauuaaacuccuuuggguagcugugauuggagacuggcucaaccucgucuuuaaguggauucucuuuggacagcguccauacugguggguuuuggauacugacuacuacagcaacacuuccgugccccugauaaagcaguucccuguaaccugugagacuggaccagggagccccucuggccaugccaugggcacagcagguguauacuacgugauggucacaucuacucuuuccaucuuucagggaaagauaaagccgaccuacagauuucggugcuugaaugucauuuugugguugggauucugggcugugcagcugaaugucugucugucacgaaucuaccuugcugcucauuuuccucaucaaguuguugcuggaguccugucaggcauugcuguugcagaaacuuucagccacauccacagcaucuauaaugccagccucaagaaauauuuucucauuaccuucuuccuguucagcuucgccaucggauuuuaucugcugcucaagggacuggguguagaccuccuguggacucuggagaaagcccagagguggugcgagcagccagaauggguccacauugacaccacacccuuugccagccuccucaagaaccugggcacgcucuuuggccuggggcuggcucucaacuccagcauguacagggagagcugcaaggggaaacucagcaaguggcucccauuccgccucggcucuauuguagccucccucguccuccugcacgucuuugacuccuugaaacccccaucccaagucgagcuggucuucuacgucuuguccuucugcaagagugcgguagugccccuggcauccgucagugucauccccuacugccucgcccagguccugggccagccgcacaagaagucguug

SEQ ID NO: 16 - RNA, 1071 nt, Artificial Sequence
  source: /note="Description of Artificial Sequence: Synthetic polynucleotide"
auggaggaaggaaugaauguucuccaugacuuugggauccagucaacacauuaccuccaggugaauuaccaagacucccaggacugguucaucuugguguccgugaucgcagaccucaggaaugccuucuacguccucuuccccaucugguuccaucuucaggaagcugugggcauuaaacuccuuuggguagcugugauuggagacuggcucaaccucgucuuuaaguggauucucuuuggacagcguccauacugguggguuuuggauacugacuacuacagcaacacuuccgugccccugauaaagcaguucccuguaaccugugagacuggaccagggagccccucuggccaugccaugggcacagcagguguauacuacgugauggucacaucuacucuuuccaucuuucagggaaagauaaagccgaccuacagauuucggugcuugaaugucauuuugugguugggauucugggcugugcagcugaaugucugucugucacgaaucuaccuugcugcucauuuuccucaucaaguuguugcuggaguccugucaggcauugcuguugcagaaacuuucagccacauccacagcaucuauaaugccagccucaagaaauauuuucucauuaccuucuuccuguucagcuucgccaucggauuuuaucugcugcucaagggacuggguguagaccuccuguggacucuggagaaagcccagagguggugcgagcagccagaauggguccacauugacaccacacccuuugccagccuccucaagaaccugggcacgcucuuuggccuggggcuggcucucaacuccagcauguacagggagagcugcaaggggaaacucagcaaguggcucccauuccgccucagcuguauuguagccucccucguccuccugcacgucuuugacuccuugaaacccccaucccaagucgagcuggucuucuacgucuuguccuucugcaagagugcgguagugccccuggcauccgucagugucauccccuacugccucgcccagguccugggccagccgcacaagaagucguug

SEQ ID NO: 17 - RNA, 1071 nt, Artificial Sequence
  source: /note="Description of Artificial Sequence: Synthetic polynucleotide"
auggaggaaggaaugaauguucuccaugacuuugggauccagucaacacauuaccuccaggugaauuaccaagacucccaggacugguucaucuugguguccgugaucgcagaccucaggaaugccuucuacguccucuuccccaucugguuccaucuucaggaagcugugggcauuaaacuccuuuggguagcugugauuggagacuggcucaaccucgucuuuaaguggauucucuuuggacagcguccauacugguggguuuuggauacugacuacuacagcaacacuuccgugccccugauaaagcaguucccuguaaccugugagacuggaccagggagccccucuggccaugccaugggcacagcagguguauacuacgugauggucacaucuacucuuuccaucuuucagggaaagauaaagccgaccuacagauuucggugcuugaaugucauuuugugguugggauucugggcugugcagcugaaugucugucugucacgaaucuaccuugcugcucauuuuccucaucaaguuguugcuggaguccugucaggcauugcuguugcagaaacuuucagccacauccacagcaucuauaaugccagccucaagaaauauuuucucauuaccuucuuccuguucagcuucgccaucggauuuuaucugcugcucaagggacuggguguagaccuccuguggacucuggagaaagcccagagguggugcgagcagccagaauggguccacauugacaccacacccuuugccagccuccucaagaaccugggcacgcucuuuggccuggggcuggcucucaacuccagcauguacagggagagcugcaaggggaaacucagcaaguggcucccauuccgccucagcucuauuguagccucccucguccuccugcaccucuuugacuccuugaaacccccaucccaagucgagcuggucuucuacgucuuguccuucugcaagagugcgguagugccccuggcauccgucagugucauccccuacugccucgcccagguccugggccagccgcacaagaagucguug

SEQ ID NO: 18 - RNA, 1071 nt, Artificial Sequence
  source: /note="Description of Artificial Sequence: Synthetic polynucleotide"
auggaggaaggaaugaauguucuccaugacuuugggauccagucaacacauuaccuccaggugaauuaccaagacucccaggacugguucaucuugguguccgugaucgcagaccucaggaaugccuucuacguccucuuccccaucugguuccaucuucaggaagcugugggcauuaaacuccuuuggguagcugugauuggagacuggcucaaccucgucuuuaaguggauucucuuuggacagcguccauacugguggguuuuggauacugacuacuacagcaacacuuccgugccccugauaaagcaguucccuguaaccugugagacuggaccagggagccccucuggccaugccaugggcacagcagguguauacuacgugauggucacaucuacucuuuccaucuuucagggaaagauaaagccgaccuacagauuucggugcuugaaugucauuuugugguugggauucugggcugugcagcugaaugucugucugucacgaaucuaccuugcugcucauuuuccucaucaaguuguugcuggaguccugucaggcauugcuguugcagaaacuuucagccacauccacagcaucuauaaugccagccucaagaaauauuuucucauuaccuucuuccuguucagcuucgccaucggauuuuaucugcugcucaagggacuggguguagaccuccuguggacucuggagaaagcccagagguggugcgagcagccagaauggguccacauugacaccacacccuuugccagccuccucaagaaccugggcacgcucuuuggccuggggcuggcucucaacuccagcauguacagggagagcugcaaggggaaacucagcaaguggcucccauuccgccucagcucuauuguagccucccucguccuccugcacgucuuugacuccuugaaacccccaucccaagucgagcugaucuucuacgucuuguccuucugcaagagugcgguagugccccuggcauccgucagugucauccccuacugccucgcccagguccugggccagccgcacaagaagucguug

SEQ ID NO: 19 - RNA, 1071 nt, Artificial Sequence
  source: /note="Description of Artificial Sequence: Synthetic polynucleotide"
auggaggaaggaaugaauguucuccaugacuuugggauccagucaacacauuaccuccaggugaauuaccaagacucccaggacugguucaucuugguguccgugaucgcagaccucaggaaugccuucuacguccucuuccccaucugguuccaucuucaggaagcugugggcauuaaacuccuuuggguagcugugauuggagacuggcucaaccucgucuuuaaguggauucucuuuggacagcguccauacugguggguuuuggauacugacuacuacagcaacacuuccgugccccugauaaagcaguucccuguaaccugugagacuggaccagggagccccucuggccaugccaugggcacagcagguguauacuacgugauggucacaucuacucuuuccaucuuucagggaaagauaaagccgaccuacagauuucggugcuugaaugucauuuugugguugggauucugggcugugcagcugaaugucugucugucacgaaucuaccuugcugcucauuuuccucaucaaguuguugcuggaguccugucaggcauugcuguugcagaaacuuucagccacauccacagcaucuauaaugccagccucaagaaauauuuucucauuaccuucuuccuguucagcuucgccaucggauuuuaucugcugcucaagggacuggguguagaccuccuguggacucuggagaaagcccagagguggugcgagcagccagaauggguccacauugacaccacacccuuugccagccuccucaagaaccugggcacgcucuuuggccuggggcuggcucucaacuccagcauguacagggagagcugcaaggggaaacucagcaaguggcucccauuccgccucagcucuauuguagccucccucguccuccugcacgucuuugacuccuugaaacccccaucccaagucgagcugcucuucuacgucuuguccuucugcaagagugcgguagugccccuggcauccgucagugucauccccuacugccucgcccagguccugggccagccgcacaagaagucguug

SEQ ID NO: 20 - RNA, 1071 nt, Artificial Sequence
  source: /note="Description of Artificial Sequence: Synthetic polynucleotide"
auggaggaaggaaugaauguucuccaugacuuugggauccagucaacacauuaccuccaggugaauuaccaagacucccaggacugguucaucuugguguccgugaucgcagaccucaggaaugccuucuacguccucuuccccaucugguuccaucuucaggaagcugugggcauuaaacuccuuuggguagcugugauuggagacuggcucaaccucgucuuuaaguggauucucuuuggacagcguccauacugguggguuuuggauacugacuacuacagcaacacuuccgugccccugauaaagcaguucccuguaaccugugagacuggaccagggagccccucuggccaugccaugggcacagcagguguauacuacgugauggucacaucuacucuuuccaucuuucagggaaagauaaagccgaccuacagauuucggugcuugaaugucauuuugugguugggauucugggcugugcagcugaaugucugucugucacgaaucuaccuugcugcucauuuuccucaucaaguuguugcuggaguccugucaggcauugcuguugcagaaacuuucagccacauccacagcaucuauaaugccagccucaagaaauauuuucucauuaccuucuuccuguucagcuucgccaucggauuuuaucugcugcucaagggacuggguguagaccuccuguggacucuggagaaagcccagagguggugcgagcagccagaauggguccacauugacaccacacccuuugccagccuccucaagaaccugggcacgcucuuuggccuggggcuggcucucaacuccagcauguacagggagagcugcaaggggaaacucagcaaguggcucccauuccgccucagcucuauuguagccucccucguccuccugcacgucuuugacuccuugaaacccccaucccaagucgagcuggucuucuacgucuuguccuucugcaagagugcgguagugccccuggcauccgucagucucauccccuacugccucgcccagguccugggccagccgcacaagaagucguug

SEQ ID NO: 21 - protein, 357 aa, Artificial Sequence
  source: /note="Description of Artificial Sequence: Synthetic polypeptide"
MEEGMNILHDFGIQSTRYLQVNYQDSQDWFILVSVIADLRNAFYVLFPIWFHLKETVGINLLWVAVVGDWFNLVFKWILFGQRPYWWVLDTDYYSNSSVPIIKQFPVTCETGPGSPSGHAMGAAGVYYVMVTSTLAIFRGKKKPTYGFRCLNVILWLGFWAVQLNVCLSRIYLAAHFPHQVVAGVLSGIAVAETFSHIRGIYNASLRKYCLITIFLFGFALGFYLLLKGLGVDLLWTLEKAKRWCERPEWVHLDTTPFASLFKNLGTLLGLGLALNSSMYRKSCKGELSKLLPFRFACIVASLVLLHLFDSLKPPSQVELIFYILSFCKSATVPFASVSLIPYCLARILGQTHKKSL

SEQ ID NO: 22 - RNA, 1071 nt, Artificial Sequence
  source: /note="Description of Artificial Sequence: Synthetic polynucleotide"
auggaggaaggaaugaauguucuccaugacuuugggauccagucaacacauuaccuccaggugaauuaccaagacucccaggacugguucaucuugguguccgugaucgcagaccucaggaaugccuucuacguccucuuccccaucugguuccaucuucaggaagcugugggcauuaaacuccuuuggguagcugugauuggagacuggcucaaccucgucuuuaaguggauucucuuuggacagcguccauacugguggguuuuggauacugacuacuacagcaacacuuccgugccccugauaaagcaguucccuguaaccugugagacuggaccagggagccccucuggccaugccaugggcacagcagguguauacuacgugauggucacaucuacucuuuccaucuuucagggaaagauaaagccgaccuacagauuucggugcuugaaugucauuuugugguugggauucugggcugugcagcugaaugucugucugucacgaaucuaccuugcugcucauuuuccucaucaaguuguugcuggaguccugucaggcauugcuguugcagaaacuuucagccacauccacagcaucuauaaugccagccucaagaaauauuuucucauuaccuucuuccuguucagcuucgccaucggauuuuaucugcugcucaagggacuggguguagaccuccuguggacucuggagaaagcccagagguggugcgagcagccagaauggguccacauugacaccacacccuuugccagccuccucaagaaccugggcacgcucuuuggccuggggcuggcucucaacuccagcauguacagggagagcugcaaggggaaacucagcaaguggcucccauuccgccucagcgcuauuguagccucccucguccuccugcacgucuuugacuccuugaaacccccaucccaagucgagcuggucuucuacgucuuguccuucugcaagagugcgguagugccccuggcauccgucagugucauccccuacugccucgcccagguccugggccagccgcacaagaagucguug

SEQ ID NO: 23 - RNA, 1071 nt, Artificial Sequence
  source: /note="Description of Artificial Sequence: Synthetic polynucleotide"
auggaggagggcaugaacgugcuucacgacuucggcauccagucaacccauuaccuacaggugaacuaucaggacucccaggauugguucauccucgugagcgugaucgccgaucuaagaaacgcauucuacguguuguucccaaucugguuccaccugcaggaagcugugggcaucaagcuccuuuggguggccgugauuggcgauuggcugaaccugguguucaaguggauucucuucggucagcggccuuacugguggguguuggauaccgacuauuacaguaacaccucuguuccgcugaucaagcaguucccugucaccugcgaaaccggaccuggcuccccuuccggccacgccaugggcaccgccggcguguacuacgugauggugacauccacccugagcaucuuccagggcaagaucaagccuaccuacagauucaggugccugaacguuaucuuguggcugggauucugggcagugcagcucaacgugugccugagcaggaucuaucucgcagcccacuucccacaucaggucguggccggcguacugagcggaaucgccguggcugaaaccuucagccauauccacagcaucuacaaugccucccugaagaaguacuuccuuauuacauucuuccuguucucuuucgccaucggcuucuaucugcugcuaaagggccugggcgucgaccuccuguggacccuggagaaggcccagagauggugcgaacaaccugagugggugcacaucgacaccacuccguucgcuagccugcucaagaaccugggcacucuuuucggccugggccuggcccucaauagcagcauguaccgggagagcuguaagggaaagcuguccaaguggcucccuuucagacuuagcugcaucguggcgucucucgugcugcugcacguguucgacagccugaagccuccuucgcagguggagcugguguucuacgugcugagcuucugcaagagcgcgguggugccacuggcaagugucagcgugaucccuuauugccuggcccaggugcugggccagccucauaagaagucccug

SEQ ID NO: 24 - RNA, 1071 nt, Artificial Sequence
  source: /note="Description of Artificial Sequence: Synthetic polynucleotide"
auggaggagggcaugaacgugcuucacgacuucggcauccagucaacccauuaccuacaggugaacuaucaggacucccaggauugguucauccucgugagcgugaucgccgaucuaagaaacgcauucuacguguuguucccaaucugguuccaccugcaggaagcugugggcaucaagcuccuuuggguggccgugauuggcgauuggcugaaccugguguucaaguggauucucuucggucagcggccuuacugguggguguuggauaccgacuauuacaguaacaccucuguuccgcugaucaagcaguucccugucaccugcgaaaccggaccuggcuccccuuccggccacgccaugggcaccgccggcguguacuacgugauggugacauccacccugagcaucuucaggggcaagaucaagccuaccuacagauucaggugccugaacguuaucuuguggcugggauucugggcagugcagcucaacgugugccugagcaggaucuaucucgcagcccacuucccacaucaggucguggccggcguacugagcggaaucgccguggcugaaaccuucagccauauccacagcaucuacaaugccucccugaagaaguacuuccuuauuacauucuuccuguucucuuucgccaucggcuucuaucugcugcuaaagggccugggcgucgaccuccuguggacccuggagaaggcccagagauggugcgaacggccugagugggugcacaucgacaccacuccguucgcuagccugcucaagaaccugggcacucuuuucggccugggccuggcccucaauagcagcauguaccgggagagcuguaagggaaagcuguccaaguggcucccuuucagacuuagcugcaucguggcgucucucgugcugcugcacguguucgacagccugaagccuccuucgcagguggagcugguguucuacgugcugagcuucugcaagagcgcgguggugccacuggcaagugucagcgugaucccuuauugccuggcccaggugcugggccagccucauaagaagucccug

SEQ ID NO: 25 - RNA, 1071 nt, Artificial Sequence
  source: /note="Description of Artificial Sequence: Synthetic polynucleotide"
auggaggagggcaugaacgugcuucacgacuucggcauccagucaacccauuaccuacaggugaacuaucaggacucccaggauugguucauccucgugagcgugaucgccgaucuaagaaacgcauucuacguguuguucccaaucugguuccaccugcaggaagcugugggcaucaagcuccuuuggguggccgugauuggcgauuggcugaaccugguguucaaguggauucucuucggucagcggccuuacugguggguguuggauaccgacuauuacaguaacaccucuguuccgcugaucaagcaguucccugucaccugcgaaaccggaccuggcuccccuuccggccacgccaugggcaccgccggcguguacuacgugauggugacauccacccugagcaucuucaggggcaagaagaagccuaccuacagauucaggugccugaacguuaucuuguggcugggauucugggcagugcagcucaacgugugccugagcaggaucuaucucgcagcccacuucccacaucaggucguggccggcguacugagcggaaucgccguggcugaaaccuucagccauauccacagcaucuacaaugccucccugaagaaguacuuccuuauuacauucuuccuguucucuuucgccaucggcuucuaucugcugcuaaagggccugggcgucgaccuccuguggacccuggagaaggcccagagauggugcgaacggccugagugggugcacaucgacaccacuccguucgcuagccugcucaagaaccugggcacucuuuucggccugggccuggcccucaauagcagcauguaccgggagagcuguaagggaaagcuguccaaguggcucccuuucagacuuggaugcaucguggcgucucucgugcugcugcaccuguucgacagccugaagccuccuucgcagguggagcugauuuucuacgugcugagcuucugcaagagcgcgguggugccacuggcaagugucagccugaucccuuauugccuggcccaggugcugggccagccucauaagaagucccug

SEQ ID NO: 26 - RNA, 1071 nt, Artificial Sequence
  source: /note="Description of Artificial Sequence: Synthetic polynucleotide"
auggaggagggcaugaacguacuucacgacuucggcauccagagcacccacuacuugcaggugaacuaccaggacucccaggauugguucauucucgugagcgugauugccgaucuccggaacgcuuucuacgugcuguucccuauuugguuccaccugcaggaggcugugggcaucaaguugcugugggucgccgugauaggcgacuggcucaacuugguguucaaguggauucuguucggccagcguccauacuggugggugcuggacacagacuauuauucuaauacaagcguaccucugaucaagcaguucccagugaccugcgaaacgggaccuggaucaccaagcggccacgccaugggaacggcuggcguguacuacgugauggugaccagcacccucagcaucuuccagggaaagaucaagccgacuuacagauuccguugccugaacgugauccuguggcucggauucugggccgugcagcucaacgugugccugaguagaaucuaccuggccgcucacuucccucaccagguaguggccggcgugcugagcggcauugccguggccgagacauucagucacauccacagcaucuauaacgcuagccugaagaaguauuuccugauuacauucuuccuguucucuuucgcuaucggcuucuaccuccuccugaagggccugggcguggaccuguuguggacccuggagaaggcucagagguggugcgagcaaccugaguggguccauaucgauaccaccccauucgcaagucugcugaagaaccugggcacacucuucggccugggccuggcccugaacagcucgauguacagagagucuugcaagggaaagcuuagcaaguggcucccuuucagacugucuugcaucguggccagccuggugcugcugcauguguucgacucucugaagccuccuucacaggucgagcugguuuucuaugugcugaguuucugcaaguccgcuguggugccucuggcuagcgugagcgugaucccuuacugccuggcccaggugcugggccagccucacaagaagucccua

SEQ ID NO: 27 - RNA, 1071 nt, Artificial Sequence
  source: /note="Description of Artificial Sequence: Synthetic polynucleotide"
auggaggagggcaugaacguacuucacgacuucggcauccagagcacccacuacuugcaggugaacuaccaggacucccaggauugguucauucucgugagcgugauugccgaucuccggaacgcuuucuacgugcuguucccuauuugguuccaccugcaggaggcugugggcaucaaguugcugugggucgccgugauaggcgacuggcucaacuugguguucaaguggauucuguucggccagcguccauacuggugggugcuggacacagacuauuauucuaauacaagcguaccucugaucaagcaguucccagugaccugcgaaacgggaccuggaucaccaagcggccacgccaugggaacggcuggcguguacuacgugauggugaccagcacccucagcaucuuccggggaaagaucaagccgacuuacagauuccguugccugaacgugauccuguggcucggauucugggccgugcagcucaacgugugccugaguagaaucuaccuggccgcucacuucccucaccagguaguggccggcgugcugagcggcauugccguggccgagacauucagucacauccacagcaucuauaacgcuagccugaagaaguauuuccugauuacauucuuccuguucucuuucgcuaucggcuucuaccuccuccugaagggccugggcguggaccuguuguggacccuggagaaggcucagagguggugcgagaggccugaguggguccauaucgauaccaccccauucgcaagucugcugaagaaccugggcacacucuucggccugggccuggcccugaacagcucgauguacagagagucuugcaagggaaagcuuagcaaguggcucccuuucagacugucuugcaucguggccagccuggugcugcugcauguguucgacucucugaagccuccuucacaggucgagcugguuuucuaugugcugaguuucugcaaguccgcuguggugccucuggcuagcgugagcgugaucccuuacugccuggcccaggugcugggccagccucacaagaagucccua

SEQ ID NO: 28 - RNA, 1071 nt, Artificial Sequence
  source: /note="Description of Artificial Sequence: Synthetic polynucleotide"
auggaggagggcaugaacguacuucacgacuucggcauccagagcacccacuacuugcaggugaacuaccaggacucccaggauugguucauucucgugagcgugauugccgaucuccggaacgcuuucuacgugcuguucccuauuugguuccaccugcaggaggcugugggcaucaaguugcugugggucgccgugauaggcgacuggcucaacuugguguucaaguggauucuguucggccagcguccauacuggugggugcuggacacagacuauuauucuaauacaagcguaccucugaucaagcaguucccagugaccugcgaaacgggaccuggaucaccaagcggccacgccaugggaacggcuggcguguacuacgugauggugaccagcacccucagcaucuuccggggaaagaagaagccgacuuacagauuccguugccugaacgugauccuguggcucggauucugggccgugcagcucaacgugugccugaguagaaucuaccuggccgcucacuucccucaccagguaguggccggcgugcugagcggcauugccguggccgagacauucagucacauccacagcaucuauaacgcuagccugaagaaguauuuccugauuacauucuuccuguucucuuucgcuaucggcuucuaccuccuccugaagggccugggcguggaccuguuguggacccuggagaaggcucagagguggugcgagaggccugaguggguccauaucgauaccaccccauucgcaagucugcugaagaaccugggcacacucuucggccugggccuggcccugaacagcucgauguacagagagucuugcaagggaaagcuuagcaaguggcucccuuucagacugggaugcaucguggccagccuggugcugcugcaucuguucgacucucugaagccuccuucacaggucgagcugauuuucuaugugcugaguuucugcaaguccgcuguggugccucuggcuagcgugagccugaucccuuacugccuggcccaggugcugggccagccucacaagaagucccua

SEQ ID NO: 29 - RNA, 1071 nt, Artificial Sequence
  source: /note="Description of Artificial Sequence: Synthetic polynucleotide"
auggaggaaggaaugaacgugcuucacgauuucggcauucaaagcacccauuaccuccaggugaacuaccaggacagccaggacugguucauuuuggucagcguaauugccgaucucaggaacgcauucuacgugcuguucccuaucugguuccaccugcaggaagccgugggcauuaagcugcuuuggguggccgugaucggcgacuggcugaaccugguguucaaguggauccuguucggccagcggccauacuggugggugcuggauaccgacuacuacagcaacacuucugucccgcugauaaagcaguucccgguaacgugcgaaacgggcccuggcagcccuagcggacacgccaugggcaccgccggcguguacuacgugauggugacuucgacccucagcauuuuccagggaaagaucaagccaaccuacagauucaggugucucaaugugauucuguggcugggcuucugggcugugcaguugaacgugugccucagcagaauuuaccuggccgcccacuucccucaccaggugguggccggugugcugagcggcauugcuguggccgagacguucucgcauauccacagcaucuacaacgccagcuuaaagaaguacuuccugaucaccuucuuccucuucuccuucgcuaucggauucuaucugcugcugaagggacugggcgucgaccugcuguggacgcuggagaaggcccagcgguggugcgagcagccagagugggugcauaucgauacuaccccauucgccucucuguuaaagaaccugggcacacuguucggucugggccuggcccucaacuccagcauguaccgggagagcugcaagggaaagcuguccaaguggcugccuuuccgccugggcugcaucguggcuagccuuguccugcugcaucucuucgacagccucaagccuccaagccagguggaacugauuuucuacgugcugagcuucugcaagucagcuguggugccacuggcuagcgugucacugauuccuuacugccucgcccaggucuuaggccagccucauaagaagucgcug

SEQ ID NO: 30 - RNA, 1071 nt, Artificial Sequence
  source: /note="Description of Artificial Sequence: Synthetic polynucleotide"
auggaggagggaaugaacgucuuacacgacuucggcauccaguccacccacuaccuacaggugaauuaccaggacagccaagauugguucauccucgugagcguuauagccgacuugagaaacgccuucuacguguuguucccaaucugguuccaccuccaggaggcaguuggaauuaagcugcuguggguggcagugaucggcgacuggcugaaccuggucuucaaguggauuuuguucggccagaggccuuacuggugggugcuggauacagacuacuacuccaacacaagcgugccgcugauuaagcaguucccugugaccugugagacaggcccuggcuccccaagcggccacgccaugggcacagccgguguguacuacguuauggugacuagcacgcugucgauuuuccagggcaagaucaagccaaccuacagauucaggugccugaaugugauccuguggcucggcuucugggccguccagcugaacgugugccugagccgcaucuaucuggcggcucacuucccacaccaagugguugccggagugcucagcggcaucgcagucgccgaaaccuucagccacauucacagcauuuauaaugcuagccugaagaaguauuuccugaucaccuucuuccucuucagcuucgccauuggcuucuaucugcugcucaagggccugggcguggaccuucuguggacacuggagaaggcucagcgcuggugcgaacagccagagugggugcacaucgacaccaccccguucgccucccugcugaagaaucugggcacccuguucggccucggccuggcccugaacaguagcauguacagggaaagcuguaagggcaagcugagcaaguggcucccauuccggcugggcugcaucguugccagccuggugcugcugcaccuuuucgacucccugaagccaccuucacagguggagcucaucuucuacgugcucuccuucugcaaguccgcuguggugccgcuggcgagugugagccugaucccauacugccuugcccaggugcugggucagccucauaagaaguccuug

SEQ ID NO: 31 - RNA, 1071 nt, Artificial Sequence
  source: /note="Description of Artificial Sequence: Synthetic polynucleotide"
auggaggagggcaugaacgugcuucacgacuucggcauccagucaacccauuaccuacaggugaacuaucaggacucccaggauugguucauccucgugagcgugaucgccgaucuaagaaacgcauucuacguguuguucccaaucugguuccaccugcaggaagcugugggcaucaagcuccuuuggguggccgugauuggcgauuggcugaaccugguguucaaguggauucucuucggucagcggccuuacugguggguguuggauaccgacuauuacaguaacaccucuguuccgcugaucaagcaguucccugucaccugcgaaaccggaccuggcuccccuuccggccacgccaugggcaccgccggcguguacuacgugauggugacauccacccugagcaucuuccagggcaagaucaagccuaccuacagauucaggugccugaacguuaucuuguggcugggauucugggcagugcagcucaacgugugccugagcaggaucuaucucgcagcccacuucccacaucaggucguggccggcguacugagcggaaucgccguggcugaaaccuucagccauauccacagcaucuacaaugccucccugaagaaguacuuccuuauuacauucuuccuguucucuuucgccaucggcuucuaucugcugcuaaagggccugggcgucgaccuccuguggacccuggagaaggcccagagauggugcgaacaaccugagugggugcacaucgacaccacuccguucgcuagccugcucaagaaccugggcacucuuuucggccugggccuggcccucaauagcagcauguaccgggagagcuguaagggaaagcuguccaaguggcucccuuucagacuuggaugcaucguggcgucucucgugcugcugcaccuguucgacagccugaagccuccuucgcagguggagcugauuuucuacgugcugagcuucugcaagagcgcgguggugccacuggcaagugucagccugaucccuuauugccuggcccaggugcugggccagccucauaagaagucccug

SEQ ID NO: 32 - RNA, 1071 nt, Artificial Sequence
  source: /note="Description of Artificial Sequence: Synthetic polynucleotide"
auggaggagggcaugaacgugcuccacgacuucggcauccagagcacccacuaccuccaggugaacuaccaggacagccaggacugguucauccucgugagcgugaucgccgacuugcggaacgccuucuacguguuguuccccaucugguuccacuugcaggaggccgugggcaucaagcugcuguggguggccgugaucggcgacuggcugaaccugguguucaaguggauccuguucggccagcggcccuacuggugggugcuggacaccgacuacuacagcaacaccagcgugccccugaucaagcaguuccccgugaccugcgagacgggccccggcagcccuucuggucacgccaugggcaccgccggcguguacuacgugauggugaccagcacccugagcaucuuccagggcaagaucaagcccaccuaccgguuccggugccugaacgugauccuguggcugggcuucugggccgugcagcugaaugugugccugagccggaucuaccuggccgcccacuucccacaccaggugguggccggcguccugagcggcaucgccguggccgagacguucagccacauccacagcaucuacaacgccagccugaagaaguacuuccugaucaccuucuuccuguucagcuucgccaucggcuucuaccugcugcugaagggccugggcguggaccuucuguggacccuggagaaggcccagcgguggugcgagcagcccgagugggugcacaucgacaccaccccauucgcaagccugcuaaagaaccugggcacacucuucggccugggacuggcccugaacagcagcauguaccgggagagcugcaagggcaagcugagcaaguggcugcccuucaggcuuggcugcaucguggcuagccuggugcugcugcaccuguucgacucccugaagccucccagccagguggagcugaucuucuauguccucagcuucugcaagagcgccguggugccacucgccagcgugagccugauccccuacugccuggcccaggugcugggccagccccacaagaagucccug

SEQ ID NO: 33 - RNA, 1071 nt, Artificial Sequence
  source: /note="Description of Artificial Sequence: Synthetic polynucleotide"
auggaggagggcaugaacgugcuccacgacuucggcauccagagcacccacuaccuccaggugaacuaccaggacagccaggacugguucaucuuggugagcgugaucgccgacuugcggaacgccuucuacgugcuguuccccaucugguuccaccugcaagaggccgugggcaucaagcugcuguggguggccgugaucggcgacuggcugaaccugguguucaaguggauccuguucggccagcggcccuacuggugggugcuggacaccgacuacuacagcaacaccagcgugccccugaucaagcaguuccccgugaccugcgagacuggccccggcagcccuagcggacacgccaugggcaccgccggcguguacuacgugauggugaccagcacccugagcaucuuccagggcaagaucaagcccaccuaccgguuccggugccugaacgugauccuguggcugggcuucugggccgugcagcucaaugucugccugagccggaucuaccuggccgcccacuucccucaccaggugguggccggaguucugagcggcaucgccguggccgagacuuucagccacauccacagcaucuacaacgccagccugaagaaguacuuccugaucaccuucuuccuguucagcuucgccaucggcuucuaccugcugcugaagggccugggcguggaccuucuguggacccuggagaaggcccagcgguggugcgagcagcccgagugggugcacaucgacaccacaccuuucgccucacugcucaagaaccugggcacgcuguucggacugggccuggcccugaacagcagcauguaccgggagagcugcaagggcaagcugagcaaguggcugcccuucagacugggaugcaucguggcgagcuuggugcugcugcaccuguucgauucccugaagccacccagccagguggagcugaucuucuauguccucagcuucuguaagagcgccguggugccgcuggccagcgugagccugauccccuacugucuggcccaggugcugggccagccccacaagaagucccug

SEQ ID NO: 34 - RNA, 1071 nt, Artificial Sequence
  source: /note="Description of Artificial Sequence: Synthetic polynucleotide"
auggaggagggcaugaacguacuucacgacuucggcauccagagcacccacuacuugcaggugaacuaccaggacucccaggauugguucauucucgugagcgugauugccgaucuccggaacgcuuucuacgugcuguucccuauuugguuccaccugcaggaggcugugggcaucaaguugcugugggucgccgugauaggcgacuggcucaacuugguguucaaguggauucuguucggccagcguccauacuggugggugcuggacacagacuauuauucuaauacaagcguaccucugaucaagcaguucccagugaccugcgaaacgggaccuggaucaccaagcggccacgccaugggaacggcuggcguguacuacgugauggugaccagcacccucagcaucuuccggggaaagaagaagccgacuuacagauuccguugccugaacgugauccuguggcucggauucugggccgugcagcucaacgugugccugaguagaaucuaccuggccgcucacuucccucaccagguaguggccggcgugcugagcggcauugccguggccgagacauucagucacauccacagcaucuauaacgcuagccugaagaaguauuuccugauuacauucuuccuguucucuuucgcuaucggcuucuaccuccuccugaagggccugggcguggaccuguuguggacccuggagaaggcucagagguggugcgagaggccugaguggguccauaucgauaccaccccauucgcaagucugcugaagaaccugggcacacucuucggccugggccuggcccugaacagcucgauguacagagagucuugcaagggaaagcuuagcaaguggcucccuuucagacugucuugcaucguggccagccuggugcugcugcaucuguucgacucucugaagccuccuucacaggucgagcugguuuucuaugugcugaguuucugcaaguccgcuguggugccucuggcuagcgugagcgugaucccuuacugccuggcccaggugcugggccagccucacaagaagucccua

SEQ ID NO: 35 - RNA, 1071 nt, Artificial Sequence
  source: /note="Description of Artificial Sequence: Synthetic polynucleotide"
auggaggagggcaugaacguccuucacgacuucgguauccagucgacccacuaccuccaagugaacuaucaggauagccaggacugguucauuuuggugagcguaauagccgaccucagaaacgccuucuacguguuauucccuaucugguuccaccugcaggaggccgugggaauaaagcuucuuuggguggcugugauuggcgauuggcugaaccugguguucaaguggauccuguucggccagaggccauacugguggguccuggauaccgacuacuacagcaacacaagcgugccacugauuaagcaguucccggugacaugcgaaacaggcccuggcuccccuagcggccaugcuaugggcaccgccggcguguauuacgugauggugaccagcaccuugucuaucuuccgaggcaagaagaagccuaccuacagauucaggugccugaacgugauccucuggcugggcuucugggccgugcagcuaaacguuugccucuccagaaucuaccucgccgcccauuucccacaccaggugguggccggcguucugaguggcaucgccguggcugagacauucagccacauccauagcauuuacaacgccagcuugaagaaguauuuccugauuaccuucuuccuguucagcuucgccauaggcuucuaucuucuucugaagggccugggcguggaccugcuguggacccuggagaaggcccagcgguggugcgagaggccugaaugggugcauaucgauacaaccccuuucgccucccuacucaagaaccucggcacucuguucggccucggccucgcccugaacagcuccauguacagagagagcugcaagggcaagcucagcaaguggcugccauuccggcugagcugcauuguugccagccucgugcuccugcaccuguucgacagucucaagccuccuagucagguggagcugguguucuauguccugucauucugcaaguccgccguggugccucuggcuagcgugagcgucaucccauacugccuggcccaagugcugggacagccacacaagaagucguua

SEQ ID NO: 36 - RNA, 1071 nt, Artificial Sequence
  source: /note="Description of Artificial Sequence: Synthetic polynucleotide"
auggaggaggguaugaacguccuacacgacuucggcauacagucuacccacuaucuucagguuaacuaccaggacagccaggacugguucauccuugugagcguuaucgccgaccuucgcaacgcguucuacgugcuuuucccuaucugguuccaccugcaggaggcuguaggcauuaagcugcugugggucgccgugaucggcgacuggcugaaucugguguucaaguggauccuguucggccaacgcccuuauugguggguccuggacacagauuacuauucaaauaccagcgugccauugauuaagcaguucccuguuaccugcgaaaccggcccuggcuccccuuccggccaugcaaugggaaccgccggcguguacuaugucauggugaccagcacccuuucaauuuuccggggcaagaagaagccuacuuacagguucagaugccugaacgugauccuguggcugggcuucugggccgugcagcucaacgugugccugagcagaaucuaucucgccgcucacuucccucaucagguggucgccggagugcucucaggcaucgccguggcggagacguucucccacauacacagcauuuacaacgcaagccugaagaaguacuuccugaucaccuucuuccuguucagcuucgccaucggauucuaccugcugcugaagggccucggcguugaccugcuguggacccuggagaaggcccagagauggugugagcguccugagugggugcacauugacaccacuccguucgcuagccugcugaagaaccugggcacccuguucggccugggacuggcucugaacagcagcauguauagggaguccugcaagggcaagcuaucaaaguggcugccuuuccggcugagcugcauuguggccagccuggugcugcugcaccuguucgacucccugaagccgccuucccagguggagcuggucuucuacgugcuuagcuucuguaagagcgccguggugccacucgcuagcgugucuguuaucccuuacugccuggcccaggugcugggccagccucauaagaagucucuc

SEQ ID NO: 37 - RNA, 1071 nt, Artificial Sequence
  source: /note="Description of Artificial Sequence: Synthetic polynucleotide"
auggaggagggcaugaacgugcuucacgauuucggaauucagagcacccacuacuugcaggugaacuaccaggacucucaagacugguucauccuugugagcgugaucgccgaucucaggaacgccuucuacguguuguucccgauuugguuccaccuucaggaggccgucggcaucaagcugcuguggguggccgugaucggcgacuggcugaacuugguguucaaguggauucuguucggacagaggccauacuggugggugcuggacacugacuauuauaguaacacuagcgucccacugauaaagcaauucccugugaccugcgagacaggcccuggcagcccuuccggccacgccaugggcacugccggaguauacuaugugauggugaccagcacccugagcaucuucaggggaaagaagaagccuacguacagauucagaugccugaacgugauccuguggcugggcuucugggccgugcaacugaaugugugccucuccaggauuuaccuggcagcgcacuucccucaccaggucguggcuggagugcugucuggaaucgccguggccgaaacauucagccacauucacucaauuuacaaugccagccugaagaaguacuuccugaucaccuucuuccuguucaguuucgccauagguuucuaccugcugcucaagggccuaggcguugaccugcuguggacauuggagaaggcacagcgcuggugcgagaggccagaaugggugcacauugacacaaccccuuucgccagccuccugaagaaucucggcacccuguucggccugggccuggcccugaacagcucaauguauagagagagcugcaaggguaagcugagcaaguggcugccuuucaggcugagcugcaucguugccagccucguacugcuccaccucuucgacucucugaagccaccaagucagguggagcugguguucuaugugcuuagcuucugcaagagcgccguggugccucuggccagcguguccgugaucccuuacugccuggcccagguccugggccagccgcauaagaagucucug

SEQ ID NO: 38 - RNA, 1071 nt, Artificial Sequence
  source: /note="Description of Artificial Sequence: Synthetic polynucleotide"
auggaggagggcaugaacguguuacacgacuucggcauccagagcacccacuaccuccaggugaacuaccaggacagccaggacugguucauccuagugagcgugaucgccgacuuacggaacgccuucuacgugcuuuuccccaucugguuccaccuucaggaggccgugggcaucaagcugcuguggguggccgugaucggcgacuggcugaaccugguguucaaguggauccuguucggccagcggcccuacuggugggugcuggacaccgacuacuacagcaacaccagcgugccccugaucaagcaguuccccgugaccugcgagacaggccccggcagcccgagcggccacgccaugggcaccgccggcguguacuacgugauggugaccagcacccugagcaucuuccggggcaagaagaagcccaccuaccgguuccggugccugaacgugauccuguggcugggcuucugggccgugcagcuuaacgucugccugagccggaucuaccuggccgcccacuucccucaccaggugguggcuggagugcugagcggcaucgccguggccgagacauucagccacauccacagcaucuacaacgccagccugaagaaguacuuccugaucaccuucuuccuguucagcuucgccaucggcuucuaccugcugcugaagggccugggcguggaccugcucuggacccuggagaaggcccagcgguggugcgaaagacccgagugggugcacaucgacaccaccccuuucgccucucugcucaagaaccugggcacgcuuuucggucugggccuggcccugaacagcagcauguaccgggagagcugcaagggcaagcugagcaaguggcugcccuuccggcugagcugcaucguggcuagccuggugcugcugcaccuguucgauucccugaagccucccagccagguggagcucguguucuaugugcugucauucugcaagagcgccguggugccacuggccagcgugucagugauccccuacugucuggcacaggugcugggccagccccacaagaagucucug

SEQ ID NO: 39 - RNA, 57 nt, Artificial Sequence
  source: /note="Description of Artificial Sequence: Synthetic oligonucleotide"
gggaaauaagagagaaaagaagaguaagaagaaauauaagaccccggcgccgccacc

SEQ ID NO: 40 - RNA, 54 nt, Artificial Sequence
  source: /note="Description of Artificial Sequence: Synthetic oligonucleotide"
gggaaauaagagagaaaagaagaguaagaagaaauauaagaccccggcgccacc

SEQ ID NO: 41 - RNA, 6 nt, Artificial Sequence
  source: /note="Description of Artificial Sequence: Synthetic oligonucleotide"
gccrcc

SEQ ID NO: 42 - RNA, 6 nt, Artificial Sequence
  source: /note="Description of Artificial Sequence: Synthetic oligonucleotide"
gccgcc

SEQ ID NO: 43 - RNA, 10 nt, Artificial Sequence
  source: /note="Description of Artificial Sequence: Synthetic oligonucleotide"
ccccggcgcc

SEQ ID NO: 44 - RNA, 7 nt, Artificial Sequence
  source: /note="Description of Artificial Sequence: Synthetic oligonucleotide"
ccccggc

SEQ ID NO: 45 - RNA, 1261 nt, Artificial Sequence
  source: /note="Description of Artificial Sequence: Synthetic polynucleotide"
gggaaauaagagagaaaagaagaguaagaagaaauauaagagccaccauggaggaaggaaugaauguucuccaugacuuugggauccagucaacacauuaccuccaggugaauuaccaagacucccaggacugguucaucuugguguccgugaucgcagaccucaggaaugccuucuacguccucuuccccaucugguuccaucuucaggaagcugugggcauuaaacuccuuuggguagcugugauuggagacuggcucaaccucgucuuuaaguggauucucuuuggacagcguccauacugguggguuuuggauacugacuacuacagcaacacuuccgugccccugauaaagcaguucccuguaaccugugagacuggaccagggagccccucuggccaugccaugggcacagcagguguauacuacgugauggucacaucuacucuuuccaucuuucagggaaagauaaagccgaccuacagauuucggugcuugaaugucauuuugugguugggauucugggcugugcagcugaaugucugucugucacgaaucuaccuugcugcucauuuuccucaucaaguuguugcuggaguccugucaggcauugcuguugcagaaacuuucagccacauccacagcaucuauaaugccagccucaagaaauauuuucucauuaccuucuuccuguucagcuucgccaucggauuuuaucugcugcucaagggacuggguguagaccuccuguggacucuggagaaagcccagagguggugcgagcagccagaauggguccacauugacaccacacccuuugccagccuccucaagaaccugggcacgcucuuuggccuggggcuggcucucaacuccagcauguacagggagagcugcaaggggaaacucagcaaguggcucccauuccgccucagcucuauuguagccucccucguccuccugcacgucuuugacuccuugaaacccccaucccaagucgagcuggucuucuacgucuuguccuucugcaagagugcgguagugccccuggcauccgucagugucauccccuacugccucgcccagguccugggccagccgcacaagaagucguuggacuacaaggacgacgaugacaagugauaauaggcuggagccucgguggccaugcuucuugccccuugggccuccccccagccccuccuccccuuccugcacccguacccccguggucuuugaauaaagucugagugggcggc

SEQ ID NO: 46 - RNA, 1237 nt, Artificial Sequence
  source: /note="Description of Artificial Sequence: Synthetic polynucleotide"
gggaaauaagagagaaaagaagaguaagaagaaauauaagagccaccauggaggaaggaaugaacauucuccaugacuuugggauccagucgacucgcuaucuccaagugaauuaccaagacucccaggacugguucauccuugugucugugauugcugaccugaggaacgccuucuauguccucuuucccaucugguuccaucuuaaagagacugugggcaucaaucuccucuggguggcaguggucggagacugguucaaccucgucuucaaguggauucuguuuggacaacgcccguauugguggguccuggacaccgacuacuacagcaacagcuccgugccuauaauaaagcaguucccugucaccugugagaccggaccaggaagucccucuggccaugccaugggcgcagcagguguauacuauguuauggucacuucuacucuugcuaucuuucgaggaaagaaaaagccaacguauggauuccgguguuugaacgucaucuugugguugggauucugggcugugcagcugaacgucugucugucccggaucuaccuugcugcucacuuuccccaccaggucguggcuggagucuugucaggcauugcuguggcugaaacuuucagccacauccggggcaucuacaaugccagccuccggaaguauugucucaucaccaucuucuuguuugguuucgcgcuuggauucuaccugcuacuaaaagggcuagggguggaccuccuguggacuuuggagaaagcuaagagauggugugagcggccagaauggguccaccuugacacuacacccuuugccagccucuucaaaaaccugggaacccucuugggguuggggcuggcccucaacuccagcauguaccggaagagcugcaagggagaacucagcaaguugcucccauuccgcuucgccugcauuguggcuuccuugguccuccugcaucucuuugacucucugaagcccccaucccagguugaguugaucuucuacaucuugucuuucugcaagagcgcaacaguucccuuugcaucugucagucuuaucccauacugccuagcccggauccugggacagacacacaagaagucuuugugauaauaggcuggagccucgguggccaugcuucuugccccuugggccuccccccagccccuccuccccuuccugcacccguacccccguggucuuugaauaaagucugagugggcggc

SEQ ID NO: 47 - RNA, 1261 nt, Artificial Sequence
  source: /note="Description of Artificial Sequence: Synthetic polynucleotide"
gggaaauaagagagaaaagaagaguaagaagaaauauaagagccaccauggaggaaggaaugaacauucuccaugacuuugggauccagucgacucgcuaucuccaagugaauuaccaagacucccaggacugguucauccuugugucugugauugcugaccugaggaacgccuucuauguccucuuucccaucugguuccaucuuaaagagacugugggcaucaaucuccucuggguggcaguggucggagacugguucaaccucgucuucaaguggauucuguuuggacaacgcccguauugguggguccuggacaccgacuacuacagcaacagcuccgugccuauaauaaagcaguucccugucaccugugagaccggaccaggaagucccucuggccaugccaugggcgcagcagguguauacuauguuauggucacuucuacucuugcuaucuuucgaggaaagaaaaagccaacguauggauuccgguguuugaacgucaucuugugguugggauucugggcugugcagcugaacgucugucugucccggaucuaccuugcugcucacuuuccccaccaggucguggcuggagucuugucaggcauugcuguggcugaaacuuucagccacauccggggcaucuacaaugccagccuccggaaguauugucucaucaccaucuucuuguuugguuucgcgcuuggauucuaccugcuacuaaaagggcuagggguggaccuccuguggacuuuggagaaagcuaagagauggugugagcggccagaauggguccaccuugacacuacacccuuugccagccucuucaaaaaccugggaacccucuugggguuggggcuggcccucaacuccagcauguaccggaagagcugcaagggagaacucagcaaguugcucccauuccgcuucgccugcauuguggcuuccuugguccuccugcaucucuuugacucucugaagcccccaucccagguugaguugaucuucuacaucuugucuuucugcaagagcgcaacaguucccuuugcaucugucagucuuaucccauacugccuagcccggauccugggacagacacacaagaagucuuuggacuacaaggacgacgaugacaagugauaauaggcuggagccucgguggccaugcuucuugccccuugggccuccccccagccccuccuccccuuccugcacccguacccccguggucuuugaauaaagucugagugggcggc

SEQ ID NO: 48 - RNA, 1237 nt, Artificial Sequence
  source: /note="Description of Artificial Sequence: Synthetic polynucleotide"
gggaaauaagagagaaaagaagaguaagaagaaauauaagagccaccauggaggaaggaaugaauguucuccaugacuuugggauccagucaacacauuaccuccaggugaauuaccaagacucccaggacugguucaucuugguguccgugaucgcagaccucaggaaugccuucuacguccucuuccccaucugguuccaucuucaggaagcugugggcauuaaacuccuuuggguagcugugauuggagacuggcucaaccucgucuuuaaguggauucucuuuggacagcguccauacugguggguuuuggauacugacuacuacagcaacacuuccgugccccugauaaagcaguucccuguaaccugugagacuggaccagggagccccucuggccaugccaugggcacagcagguguauacuacgugauggucacaucuacucuuuccaucuuucagggaaagauaaagccgaccuacagauuucggugcuugaaugucauuuugugguugggauucugggcugugcagcugaaugucugucugucacgaaucuaccuugcugcucauuuuccucaucaaguuguugcuggaguccugucaggcauugcuguugcagaaacuuucagccacauccacagcaucuauaaugccagccucaagaaauauuuucucauuaccuucuuccuguucagcuucgccaucggauuuuaucugcugcucaagggacuggguguagaccuccuguggacucuggagaaagcccagagguggugcgagcagccagaauggguccacauugacaccacacccuuugccagccuccucaagaaccugggcacgcucuuuggccuggggcuggcucucaacuccagcauguacagggagagcugcaaggggaaacucagcaaguggcucccauuccgccucagcucuauuguagccucccucguccuccugcacgucuuugacuccuugaaacccccaucccaagucgagcuggucuucuacgucuuguccuucugcaagagugcgguagugccccuggcauccgucagugucauccccuacugccucgcccagguccugggccagccgcacaagaagucguugugauaauaggcuggagccucgguggccaugcuucuugccccuugggccuccccccagccccuccuccccuuccugcacccguacccccguggucuuugaauaaagucugagugggcggc

SEQ ID NO: 49 - RNA, 1237 nt, Artificial Sequence; identical to SEQ ID NO: 48
  source: /note="Description of Artificial Sequence: Synthetic polynucleotide"

SEQ ID NO: 50 - RNA, 1237 nt, Artificial Sequence
  source: /note="Description of Artificial Sequence: Synthetic polynucleotide"
gggaaauaagagagaaaagaagaguaagaagaaauauaagagccaccauggaggaaggaaugaauguucuccaugacuuugggauccagucaacacauuaccuccaggugaauuaccaagacucccaggacugguucaucuugguguccgugaucgcagaccucaggaaugccuucuacguccucuuccccaucugguuccaucuucaggaagcugugggcauuaaacuccuuuggguagcugugauuggagacuggcucaaccucgucuuuaaguggauucucuuuggacagcguccauacugguggguuuuggauacugacuacuacagcaacacuuccgugccccugauaaagcaguucccuguaaccugugagacuggaccagggagccccucuggccaugccaugggcacagcagguguauacuacgugauggucacaucuacucuuuccaucuuucagggaaagauaaagccgaccuacagauuucggugcuugaaugucauuuugugguugggauucugggcugugcagcugaaugucugucugucacgaaucuaccuugcugcucauuuuccucaucaaguuguugcuggaguccugucaggcauugcuguugcagaaacuuucagccacauccacagcaucuauaaugccagccucaagaaauauuuucucauuaccuucuuccuguucagcuucgccaucggauuuuaucugcugcucaagggacuggguguagaccuccuguggacucuggagaaagcccagagguggugcgagcagccagaauggguccacauugacaccacacccuuugccagccuccucaagaaccugggcacgcucuuuggccuggggcuggcucucaacuccagcauguacagggagagcugcaaggggaaacucagcaaguggcucccauuccgccucggcuguauuguagccucccucguccuccugcaccucuuugacuccuugaaacccccaucccaagucgagcugaucuucuacgucuuguccuucugcaagagugcgguagugccccuggcauccgucagucucauccccuacugccucgcccagguccugggccagccgcacaagaagucguugugauaauaggcuggagccucgguggccaugcuucuugccccuugggccuccccccagccccuccuccccuuccugcacccguacccccguggucuuugaauaaagucugagugggcggc

SEQ ID NO: 51 - RNA, 1237 nt, Artificial Sequence
  source: /note="Description of Artificial Sequence: Synthetic polynucleotide"
gggaaauaagagagaaaagaagaguaagaagaaauauaagagccaccauggaggaaggaaugaauguucuccaugacuuugggauccagucaacacauuaccuccaggugaauuaccaagacucccaggacugguucaucuugguguccgugaucgcagaccucaggaaugccuucuacguccucuuccccaucugguuccaucuucaggaagcugugggcauuaaacuccuuuggguagcugugauuggagacuggcucaaccucgucuuuaaguggauucucuuuggacagcguccauacugguggguuuuggauacugacuacuacagcaacacuuccgugccccugauaaagcaguucccuguaaccugugagacuggaccagggagccccucuggccaugccaugggcacagcagguguauacuacgugauggucacaucuacucuuuccaucuuuaggggaaagaagaagccgaccuacagauuucggugcuugaaugucauuuugugguugggauucugggcugugcagcugaaugucugucugucacgaaucuaccuugcugcucauuuuccucaucaaguuguugcuggaguccugucaggcauugcuguugcagaaacuuucagccacauccacagcaucuauaaugccagccucaagaaauauuuucucauuaccuucuuccuguucagcuucgccaucggauuuuaucugcugcucaagggacuggguguagaccuccuguggacucuggagaaagcccagagguggugcgagaggccagaauggguccacauugacaccacacccuuugccagccuccucaagaaccugggcacgcucuuuggccuggggcuggcucucaacuccagcauguacagggagagcugcaaggggaaacucagcaaguggcucccauuccgccucagcuguauuguagccucccucguccuccugcaccucuuugacuccuugaaacccccaucccaagucgagcuggucuucuacgucuuguccuucugcaagagugcgguagugccccuggcauccgucagugucauccccuacugccucgcccagguccugggccagccgcacaagaagucguugugauaauaggcuggagccucgguggccaugcuucuugccccuugggccuccccccagccccuccuccccuuccugcacccguacccccguggucuuugaauaaagucugagugggcggc

SEQ ID NO: 52 - RNA, 1237 nt, Artificial Sequence
  source: /note="Description of Artificial Sequence: Synthetic polynucleotide"
gggaaauaagagagaaaagaagaguaagaagaaauauaagagccaccauggaggaaggaaugaauguucuccaugacuuugggauccagucaacacauuaccuccaggugaauuaccaagacucccaggacugguucaucuugguguccgugaucgcagaccucaggaaugccuucuacguccucuuccccaucugguuccaucuucaggaagcugugggcauuaaacuccuuuggguagcugugauuggagacuggcucaaccucgucuuuaaguggauucucuuuggacagcguccauacugguggguuuuggauacugacuacuacagcaacacuuccgugccccugauaaagcaguucccuguaaccugugagacuggaccagggagccccucuggccaugccaugggcacagcagguguauacuacgugauggucacaucuacucuuuccaucuuucagggaaagauaaagccgaccuacagauuucggugcuugaaugucauuuugugguugggauucugggcugugcagcugaaugucugucugucacgaaucuaccuugcugcucauuuuccucaucaaguuguugcuggaguccugucaggcauugcuguugcagaaacuuucagccacauccacagcaucuauaaugccagccucaagaaauauuuucucauuaccuucuuccuguucagcuucgccaucggauuuuaucugcugcucaagggacuggguguagaccuccuguggacucuggagaaagcccagagguggugcgagcagccagaauggguccacauugacaccacacccuuugccagccuccucaagaaccugggcacgcucuuuggccuggggcuggcucucaacuccagcauguacagggagagcugcaaggggaaacucagcaaguggcucccauuccgccucagcucuauuguagccucccucguccuccugcacgucuuugacuccuugaaacccccaucccaagucgagcuggucuucuacgucuuguccuucugcaagagugcgguagugccccuggcauccgucagugucauccccuacugccucgcccagguccugggccagccgcacaagaagucguugugauaauaggcuggagccucgguggccuagcuucuugccccuugggccuccccccagccccuccuccccuuccugcacccguacccccguggucuuugaauaaagucugagugggcggc

SEQ ID NO: 53 - RNA, 1237 nt, Artificial Sequence
  source: /note="Description of Artificial Sequence: Synthetic polynucleotide"
gggaaauaagagagaaaagaagaguaagaagaaauauaagagccaccauggaggaaggaaugaauguucuccaugacuuugggauccagucaacacauuaccuccaggugaauuaccaagacucccaggacugguucaucuugguguccgugaucgcagaccucaggaaugccuucuacguccucuuccccaucugguuccaucuucaggaagcugugggcauuaaacuccuuuggguagcugugauuggagacuggcucaaccucgucuuuaaguggauucucuuuggacagcguccauacugguggguuuuggauacugacuacuacagcaacacuuccgugccccugauaaagcaguucccuguaaccugugagacuggaccagggagccccucuggccaugccaugggcacagcagguguauacuacgugauggucacaucuacucuuuccaucuuuaggggaaagauaaagccgaccuacagauuucggugcuugaaugucauuuugugguugggauucugggcugugcagcugaaugucugucugucacgaaucuaccuugcugcucauuuuccucaucaaguuguugcuggaguccugucaggcauugcuguugcagaaacuuucagccacauccacagcaucuauaaugccagccucaagaaauauuuucucauuaccuucuuccuguucagcuucgccaucggauuuuaucugcugcucaagggacuggguguagaccuccuguggacucuggagaaagcccagagguggugcgagcagccagaauggguccacauugacaccacacccuuugccagccuccucaagaaccugggcacgcucuuuggccuggggcuggcucucaacuccagcauguacagggagagcugcaaggggaaacucagcaaguggcucccauuccgccucagcucuauuguagccucccucguccuccugcacgucuuugacuccuugaaacccccaucccaagucgagcuggucuucuacgucuuguccuucugcaagagugcgguagugccccuggcauccgucagugucauccccuacugccucgcccagguccugggccagccgcacaagaagucguugugauaauaggcuggagccucgguggccuagcuucuugccccuugggccuccccccagccccuccuccccuuccugcacccguacccccguggucuuugaauaaagucugagugggcggc

SEQ ID NO: 54 - RNA, 1237 nt, Artificial Sequence
  source: /note="Description of Artificial Sequence: Synthetic polynucleotide"
gggaaauaagagagaaaagaagaguaagaagaaauauaagagccaccauggaggaaggaaugaauguucuccaugacuuugggauccagucaacacauuaccuccaggugaauuaccaagacucccaggacugguucaucuugguguccgugaucgcagaccucaggaaugccuucuacguccucuuccccaucugguuccaucuucaggaagcugugggcauuaaacuccuuuggguagcugugauuggagacuggcucaaccucgucuuuaaguggauucucuuuggacagcguccauacugguggguuuuggauacugacuacuacagcaacacuuccgugccccugauaaagcaguucccuguaaccugugagacuggaccagggagccccucuggccaugccaugggcacagcagguguauacuacgugauggucacaucuacucuuuccaucuuucagggaaagaagaagccgaccuacagauuucggugcuugaaugucauuuugugguugggauucugggcugugcagcugaaugucugucugucacgaaucuaccuugcugcucauuuuccucaucaaguuguugcuggaguccugucaggcauugcuguugcagaaacuuucagccacauccacagcaucuauaaugccagccucaagaaauauuuucucauuaccuucuuccuguucagcuucgccaucggauuuuaucugcugcucaagggacuggguguagaccuccuguggacucuggagaaagcccagagguggugcgagcagccagaauggguccacauugacaccacacccuuugccagccuccucaagaaccugggcacgcucuuuggccuggggcuggcucucaacuccagcauguacagggagagcugcaaggggaaacucagcaaguggcucccauuccgccucagcucuauuguagccucccucguccuccugcacgucuuugacuccuugaaacccccaucccaagucgagcuggucuucuacgucuuguccuucugcaagagugcgguagugccccuggcauccgucagugucauccccuacugccucgcccagguccugggccagccgcacaagaagucguugugauaauaggcuggagccucgguggccuagcuucuugccccuugggccuccccccagccccuccuccccuuccugcacccguacccccguggucuuugaauaaagucugagugggcggc

SEQ ID NO: 55 - RNA, 1237 nt, Artificial Sequence
  source: /note="Description of Artificial Sequence: Synthetic polynucleotide"
gggaaauaagagagaaaagaagaguaagaagaaauauaagagccaccauggaggaaggaaugaauguucuccaugacuuugggauccagucaacacauuaccuccaggugaauuaccaagacucccaggacugguucaucuugguguccgugaucgcagaccucaggaaugccuucuacguccucuuccccaucugguuccaucuucaggaagcugugggcauuaaacuccuuuggguagcugugauuggagacuggcucaaccucgucuuuaaguggauucucuuuggacagcguccauacugguggguuuuggauacugacuacuacagcaacacuuccgugccccugauaaagcaguucccuguaaccugugagacuggaccagggagccccucuggccaugccaugggcacagcagguguauacuacgugauggucacaucuacucuuuccaucuuucagggaaagauaaagccgaccuacagauuucggugcuugaaugucauuuugugguugggauucugggcugugcagcugaaugucugucugucacgaaucuaccuugcugcucauuuuccucaucaaguuguugcuggaguccugucaggcauugcuguugcagaaacuuucagccacauccacagcaucuauaaugccagccucaagaaauauuuucucauuaccuucuuccuguucagcuucgccaucggauuuuaucugcugcucaagggacuggguguagaccuccuguggacucuggagaaagcccagagguggugcgagaggccagaauggguccacauugacaccacacccuuugccagccuccucaagaaccugggcacgcucuuuggccuggggcuggcucucaacuccagcauguacagggagagcugcaaggggaaacucagcaaguggcucccauuccgccucagcucuauuguagccucccucguccuccugcacgucuuugacuccuugaaacccccaucccaagucgagcuggucuucuacgucuuguccuucugcaagagugcgguagugccccuggcauccgucagugucauccccuacugccucgcccagguccugggccagccgcacaagaagucguugugauaauaggcuggagccucgguggccuagcuucuugccccuugggccuccccccagccccuccuccccuuccugcacccguacccccguggucuuugaauaaagucugagugggcggc

SEQ ID NO: 56 - RNA, 1237 nt, Artificial Sequence
  source: /note="Description of Artificial Sequence: Synthetic polynucleotide"
gggaaauaagagagaaaagaagaguaagaagaaauauaagagccaccauggaggaaggaaugaauguucuccaugacuuugggauccagucaacacauuaccuccaggugaauuaccaagacucccaggacugguucaucuugguguccgugaucgcagaccucaggaaugccuucuacguccucuuccccaucugguuccaucuucaggaagcugugggcauuaaacuccuuuggguagcugugauuggagacuggcucaaccucgucuuuaaguggauucucuuuggacagcguccauacugguggguuuuggauacugacuacuacagcaacacuuccgugccccugauaaagcaguucccuguaaccugugagacuggaccagggagccccucuggccaugccaugggcacagcagguguauacuacgugauggucacaucuacucuuuccaucuuucagggaaagauaaagccgaccuacagauuucggugcuugaaugucauuuugugguugggauucugggcugugcagcugaaugucugucugucacgaaucuaccuugcugcucauuuuccucaucaaguuguugcuggaguccugucaggcauugcuguugcagaaacuuucagccacauccacagcaucuauaaugccagccucaagaaauauuuucucauuaccuucuuccuguucagcuucgccaucggauuuuaucugcugcucaagggacuggguguagaccuccuguggacucuggagaaagcccagagguggugcgagcagccagaauggguccacauugacaccacacccuuugccagccuccucaagaaccugggcacgcucuuuggccuggggcuggcucucaacuccagcauguacagggagagcugcaaggggaaacucagcaaguggcucccauuccgccucggcucuauuguagccucccucguccuccugcacgucuuugacuccuugaaacccccaucccaagucgagcuggucuucuacgucuuguccuucugcaagagugcgguagugccccuggcauccgucagugucauccccuacugccucgcccagguccugggccagccgcacaagaagucguugugauaauaggcuggagccucgguggccuagcuucuugccccuugggccuccccccagccccuccuccccuuccugcacccguacccccguggucuuugaauaaagucugagugggcggc

SEQ ID NO: 57 - RNA, 1237 nt, Artificial Sequence
  source: /note="Description of Artificial Sequence: Synthetic polynucleotide"
gggaaauaagagagaaaagaagaguaagaagaaauauaagagccaccauggaggaaggaaugaauguucuccaugacuuugggauccagucaacacauuaccuccaggugaauuaccaagacucccaggacugguucaucuugguguccgugaucgcagaccucaggaaugccuucuacguccucuuccccaucugguuccaucuucaggaagcugugggcauuaaacuccuuuggguagcugugauuggagacuggcucaaccucgucuuuaaguggauucucuuuggacagcguccauacugguggguuuuggauacugacuacuacagcaacacuuccgugccccugauaaagcaguucccuguaaccugugagacuggaccagggagccccucuggccaugccaugggcacagcagguguauacuacgugauggucacaucuacucuuuccaucuuucagggaaagauaaagccgaccuacagauuucggugcuugaaugucauuuugugguugggauucugggcugugcagcugaaugucugucugucacgaaucuaccuugcugcucauuuuccucaucaaguuguugcuggaguccugucaggcauugcuguugcagaaacuuucagccacauccacagcaucuauaaugccagccucaagaaauauuuucucauuaccuucuuccuguucagcuucgccaucggauuuuaucugcugcucaagggacuggguguagaccuccuguggacucuggagaaagcccagagguggugcgagcagccagaauggguccacauugacaccacacccuuugccagccuccucaagaaccugggcacgcucuuuggccuggggcuggcucucaacuccagcauguacagggagagcugcaaggggaaacucagcaaguggcucccauuccgccucagcuguauuguagccucccucguccuccugcacgucuuugacuccuugaaacccccaucccaagucgagcuggucuucuacgucuuguccuucugcaagagugcgguagugccccuggcauccgucagugucauccccuacugccucgcccagguccugggccagccgcacaagaagucguugugauaauaggcuggagccucgguggccuagcuucuugccccuugggccuccccccagccccuccuccccuuccugcacccguacccccguggucuuugaauaaagucugagugggcggc

SEQ ID NO: 58 - RNA, 1237 nt, Artificial Sequence
  source: /note="Description of Artificial Sequence: Synthetic polynucleotide"
gggaaauaagagagaaaagaagaguaagaagaaauauaagagccaccauggaggaaggaaugaauguucuccaugacuuugggauccagucaacacauuaccuccaggugaauuaccaagacucccaggacugguucaucuugguguccgugaucgcagaccucaggaaugccuucuacguccucuuccccaucugguuccaucuucaggaagcugugggcauuaaacuccuuuggguagcugugauuggagacuggcucaaccucgucuuuaaguggauucucuuuggacagcguccauacugguggguuuuggauacugacuacuacagcaacacuuccgugccccugauaaagcaguucccuguaaccugugagacuggaccagggagccccucuggccaugccaugggcacagcagguguauacuacgugauggucacaucuacucuuuccaucuuucagggaaagauaaagccgaccuacagauuucggugcuugaaugucauuuugugguugggauucugggcugugcagcugaaugucugucugucacgaaucuaccuugcugcucauuuuccucaucaaguuguugcuggaguccugucaggcauugcuguugcagaaacuuucagccacauccacagcaucuauaaugccagccucaagaaauauuuucucauuaccuucuuccuguucagcuucgccaucggauuuuaucugcugcucaagggacuggguguagaccuccuguggacucuggagaaagcccagagguggugcgagcagccagaauggguccacauugacaccacacccuuugccagccuccucaagaaccugggcacgcucuuuggccuggggcuggcucucaacuccagcauguacagggagagcugcaaggggaaacucagcaaguggcucccauuccgccucagcucuauuguagccucccucguccuccugcaccucuuugacuccuugaaacccccaucccaagucgagcuggucuucuacgucuuguccuucugcaagagugcgguagugccccuggcauccgucagugucauccccuacugccucgcccagguccugggccagccgcacaagaagucguugugauaauaggcuggagccucgguggccuagcuucuugccccuugggccuccccccagccccuccuccccuuccugcacccguacccccguggucuuugaauaaagucugagugggcggc

SEQ ID NO: 59 - RNA, 1237 nt, Artificial Sequence
  source: /note="Description of Artificial Sequence: Synthetic polynucleotide"
gggaaauaagagagaaaagaagaguaagaagaaauauaagagccaccauggaggaaggaaugaauguucuccaugacuuugggauccagucaacacauuaccuccaggugaauuaccaagacucccaggacugguucaucuugguguccgugaucgcagaccucaggaaugccuucuacguccucuuccccaucugguuccaucuucaggaagcugugggcauuaaacuccuuuggguagcugugauuggagacuggcucaaccucgucuuuaaguggauucucuuuggacagcguccauacugguggguuuuggauacugacuacuacagcaacacuuccgugccccugauaaagcaguucccuguaaccugugagacuggaccagggagccccucuggccaugccaugggcacagcagguguauacuacgugauggucacaucuacucuuuccaucuuucagggaaagauaaagccgaccuacagauuucggugcuugaaugucauuuugugguugggauucugggcugugcagcugaaugucugucugucacgaaucuaccuugcugcucauuuuccucaucaaguuguugcuggaguccugucaggcauugcuguugcagaaacuuucagccacauccacagcaucuauaaugccagccucaagaaauauuuucucauuaccuucuuccuguucagcuucgccaucggauuuuaucugcugcucaagggacuggguguagaccuccuguggacucuggagaaagcccagagguggugcgagcagccagaauggguccacauugacaccacacccuuugccagccuccucaagaaccugggcacgcucuuuggccuggggcuggcucucaacuccagcauguacagggagagcugcaaggggaaacucagcaaguggcucccauuccgccucagcucuauuguagccucccucguccuccugcacgucuuugacuccuugaaacccccaucccaagucgagcugaucuucuacgucuuguccuucugcaagagugcgguagugccccuggcauccgucagugucauccccuacugccucgcccagguccugggccagccgcacaagaagucguugugauaauaggcuggagccucgguggccuagcuucuugccccuugggccuccccccagccccuccuccccuuccugcacccguacccccguggucuuugaauaaagucugagugggcggc

SEQ ID NO: 60 - RNA, 1237 nt, Artificial Sequence
  source: /note="Description of Artificial Sequence: Synthetic polynucleotide"
gggaaauaagagagaaaagaagaguaagaagaaauauaagagccaccauggaggaaggaaugaauguucuccaugacuuugggauccagucaacacauuaccuccaggugaauuaccaagacucccaggacugguucaucuugguguccgugaucgcagaccucaggaaugccuucuacguccucuuccccaucugguuccaucuucaggaagcugugggcauuaaacuccuuuggguagcugugauuggagacuggcucaaccucgucuuuaaguggauucucuuuggacagcguccauacugguggguuuuggauacugacuacuacagcaacacuuccgugccccugauaaagcaguucccuguaaccugugagacuggaccagggagccccucuggccaugccaugggcacagcagguguauacuacgugauggucacaucuacucuuuccaucuuucagggaaagauaaagccgaccuacagauuucggugcuugaaugucauuuugugguugggauucugggcugugcagcugaaugucugucugucacgaaucuaccuugcugcucauuuuccucaucaaguuguugcuggaguccugucaggcauugcuguugcagaaacuuucagccacauccacagcaucuauaaugccagccucaagaaauauuuucucauuaccuucuuccuguucagcuucgccaucggauuuuaucugcugcucaagggacuggguguagaccuccuguggacucuggagaaagcccagagguggugcgagcagccagaauggguccacauugacaccacacccuuugccagccuccucaagaaccugggcacgcucuuuggccuggggcuggcucucaacuccagcauguacagggagagcugcaaggggaaacucagcaaguggcucccauuccgccucagcucuauuguagccucccucguccuccugcacgucuuugacuccuugaaacccccaucccaagucgagcugcucuucuacgucuuguccuucugcaagagugcgguagugccccuggcauccgucagugucauccccuacugccucgcccagguccugggccagccgcacaagaagucguugugauaauaggcuggagccucgguggccuagcuucuugccccuugggccuccccccagccccuccuccccuuccugcacccguacccccguggucuuugaauaaagucugagugggcggc

SEQ ID NO: 61 - RNA, 1237 nt, Artificial Sequence
  source: /note="Description of Artificial Sequence: Synthetic polynucleotide"
gggaaauaagagagaaaagaagaguaagaagaaauauaagagccaccauggaggaaggaaugaauguucuccaugacuuugggauccagucaacacauuaccuccaggugaauuaccaagacucccaggacugguucaucuugguguccgugaucgcagaccucaggaaugccuucuacguccucuuccccaucugguuccaucuucaggaagcugugggcauuaaacuccuuuggguagcugugauuggagacuggcucaaccucgucuuuaaguggauucucuuuggacagcguccauacugguggguuuuggauacugacuacuacagcaacacuuccgugccccugauaaagcaguucccuguaaccugugagacuggaccagggagccccucuggccaugccaugggcacagcagguguauacuacgugauggucacaucuacucuuuccaucuuucagggaaagauaaagccgaccuacagauuucggugcuugaaugucauuuugugguugggauucugggcugugcagcugaaugucugucugucacgaaucuaccuugcugcucauuuuccucaucaaguuguugcuggaguccugucaggcauugcuguugcagaaacuuucagccacauccacagcaucuauaaugccagccucaagaaauauuuucucauuaccuucuuccuguucagcuucgccaucggauuuuaucugcugcucaagggacuggguguagaccuccuguggacucuggagaaagcccagagguggugcgagcagccagaauggguccacauugacaccacacccuuugccagccuccucaagaaccugggcacgcucuuuggccuggggcuggcucucaacuccagcauguacagggagagcugcaaggggaaacucagcaaguggcucccauuccgccucagcucuauuguagccucccucguccuccugcacgucuuugacuccuugaaacccccaucccaagucgagcuggucuucuacgucuuguccuucugcaagagugcgguagugccccuggcauccgucagucucauccccuacugccucgcccagguccugggccagccgcacaagaagucguugugauaauaggcuggagccucgguggccuagcuucuugccccuugggccuccccccagccccuccuccccuuccugcacccguacccccguggucuuugaauaaagucugagugggcggc

SEQ ID NO: 62 - RNA, 1237 nt, Artificial Sequence
  source: /note="Description of Artificial Sequence: Synthetic polynucleotide"
gggaaauaagagagaaaagaagaguaagaagaaauauaagagccaccauggaggaaggaaugaauguucuccaugacuuugggauccagucaacacauuaccuccaggugaauuaccaagacucccaggacugguucaucuugguguccgugaucgcagaccucaggaaugccuucuacguccucuuccccaucugguuccaucuucaggaagcugugggcauuaaacuccuuuggguagcugugauuggagacuggcucaaccucgucuuuaaguggauucucuuuggacagcguccauacugguggguuuuggauacugacuacuacagcaacacuuccgugccccugauaaagcaguucccuguaaccugugagacuggaccagggagccccucuggccaugccaugggcacagcagguguauacuacgugauggucacaucuacucuuuccaucuuucagggaaagauaaagccgaccuacagauuucggugcuugaaugucauuuugugguugggauucugggcugugcagcugaaugucugucugucacgaaucuaccuugcugcucauuuuccucaucaaguuguugcuggaguccugucaggcauugcuguugcagaaacuuucagccacauccacagcaucuauaaugccagccucaagaaauauuuucucauuaccuucuuccuguucagcuucgccaucggauuuuaucugcugcucaagggacuggguguagaccuccuguggacucuggagaaagcccagagguggugcgagcagccagaauggguccacauugacaccacacccuuugccagccuccucaagaaccugggcacgcucuuuggccuggggcuggcucucaacuccagcauguacagggagagcugcaaggggaaacucagcaaguggcucccauuccgccucagcucuauuguagccucccucguccuccugcacgucuuugacuccuugaaacccccaucccaagucgagcuggucuucuacgucuuguccuucugcaagagugcggcagugccccuggcauccgucagugucauccccuacugccucgcccagguccugggccagccgcacaagaagucguugugauaauaggcuggagccucgguggccuagcuucuugccccuugggccuccccccagccccuccuccccuuccugcacccguacccccguggucuuugaauaaagucugagugggcggc

SEQ ID NO: 63 - RNA, 1237 nt, Artificial Sequence
  source: /note="Description of Artificial Sequence: Synthetic polynucleotide"
gggaaauaagagagaaaagaagaguaagaagaaauauaagagccaccauggaggaaggaaugaauguucuccaugacuuugggauccagucaacacauuaccuccaggugaauuaccaagacucccaggacugguucaucuugguguccgugaucgcagaccucaggaaugccuucuacguccucuuccccaucugguuccaucuucaggaagcugugggcauuaaacuccuuuggguagcugugauuggagacuggcucaaccucgucuuuaaguggauucucuuuggacagcguccauacugguggguuuuggauacugacuacuacagcaacacuuccgugccccugauaaagcaguucccuguaaccugugagacuggaccagggagccccucuggccaugccaugggcacagcagguguauacuacgugauggucacaucuacucuuuccaucuuuaggggaaagauaaagccgaccuacagauuucggugcuugaaugucauuuugugguugggauucugggcugugcagcugaaugucugucugucacgaaucuaccuugcugcucauuuuccucaucaaguuguugcuggaguccugucaggcauugcuguugcagaaacuuucagccacauccacagcaucuauaaugccagccucaagaaauauuuucucauuaccuucuuccuguucagcuucgccaucggauuuuaucugcugcucaagggacuggguguagaccuccuguggacucuggagaaagcccagagguggugcgagaggccagaauggguccacauugacaccacacccuuugccagccuccucaagaaccugggcacgcucuuuggccuggggcuggcucucaacuccagcauguacagggagagcugcaaggggaaacucagcaaguggcucccauuccgccucagcuguauuguagccucccucguccuccugcacgucuuugacuccuugaaacccccaucccaagucgagcuggucuucuacgucuuguccuucugcaagagugcgguagugccccuggcauccgucagugucauccccuacugccucgcccagguccugggccagccgcacaagaagucguugugauaauaggcuggagccucgguggccuagcuucuugccccuugggccuccccccagccccuccuccccuuccugcacccguacccccguggucuuugaauaaagucugagugggcggc

SEQ ID NO: 64 - RNA, 1237 nt, Artificial Sequence
  source: /note="Description of Artificial Sequence: Synthetic polynucleotide"
gggaaauaagagagaaaagaagaguaagaagaaauauaagagccaccauggaggaaggaaugaauguucuccaugacuuugggauccagucaacacauuaccuccaggugaauuaccaagacucccaggacugguucaucuugguguccgugaucgcagaccucaggaaugccuucuacguccucuuccccaucugguuccaucuucaggaagcugugggcauuaaacuccuuuggguagcugugauuggagacuggcucaaccucgucuuuaaguggauucucuuuggacagcguccauacugguggguuuuggauacugacuacuacagcaacacuuccgugccccugauaaagcaguucccuguaaccugugagacuggaccagggagccccucuggccaugccaugggcacagcagguguauacuacgugauggucacaucuacucuuuccaucuuucagggaaagauaaagccgaccuacagauuucggugcuugaaugucauuuugugguugggauucugggcugugcagcugaaugucugucugucacgaaucuaccuugcugcucauuuuccucaucaaguuguugcuggaguccugucaggcauugcuguugcagaaacuuucagccacauccacagcaucuauaaugccagccucaagaaauauuuucucauuaccuucuuccuguucagcuucgccaucggauuuuaucugcugcucaagggacuggguguagaccuccuguggacucuggagaaagcccagagguggugcgagaggccagaauggguccacauugacaccacacccuuugccagccuccucaagaaccugggcacgcucuuuggccuggggcuggcucucaacuccagcauguacagggagagcugcaaggggaaacucagcaaguggcucccauuccgccucagcuguauuguagccucccucguccuccugcacgucuuugacuccuugaaacccccaucccaagucgagcuggucuucuacgucuuguccuucugcaagagugcgguagugccccuggcauccgucagugucauccccuacugccucgcccagguccugggccagccgcacaagaagucguugugauaauaggcuggagccucgguggccuagcuucuugccccuugggccuccccccagccccuccuccccuuccugcacccguacccccguggucuuugaauaaagucugagugggcggc

SEQ ID NO: 65 - RNA, 1237 nt, Artificial Sequence
  source: /note="Description of Artificial Sequence: Synthetic polynucleotide"
gggaaauaagagagaaaagaagaguaagaagaaauauaagagccaccauggaggaaggaaugaauguucuccaugacuuugggauccagucaacacauuaccuccaggugaauuaccaagacucccaggacugguucaucuugguguccgugaucgcagaccucaggaaugccuucuacguccucuuccccaucugguuccaucuucaggaagcugugggcauuaaacuccuuuggguagcugugauuggagacuggcucaaccucgucuuuaaguggauucucuuuggacagcguccauacugguggguuuuggauacugacuacuacagcaacacuuccgugccccugauaaagcaguucccuguaaccugugagacuggaccagggagccccucuggccaugccaugggcacagcagguguauacuacgugauggucacaucuacucuuuccaucuuucagggaaagauaaagccgaccuacagauuucggugcuugaaugucauuuugugguugggauucugggcugugcagcugaaugucugucugucacgaaucuaccuugcugcucauuuuccucaucaaguuguugcuggaguccugucaggcauugcuguugcagaaacuuucagccacauccacagcaucuauaaugccagccucaagaaauauuuucucauuaccuucuuccuguucagcuucgccaucggauuuuaucugcugcucaagggacuggguguagaccuccuguggacucuggagaaagcccagagguggugcgagcagccagaauggguccacauugacaccacacccuuugccagccuccucaagaaccugggcacgcucuuuggccuggggcuggcucucaacuccagcauguacagggagagcugcaaggggaaacucagcaaguggcucccauuccgccucagcgcuauuguagccucccucguccuccugcacgucuuugacuccuugaaacccccaucccaagucgagcuggucuucuacgucuuguccuucugcaagagugcgguagugccccuggcauccgucagugucauccccuacugccucgcccagguccugggccagccgcacaagaagucguugugauaauaggcuggagccucgguggccuagcuucuugccccuugggccuccccccagccccuccuccccuuccugcacccguacccccguggucuuugaauaaagucugagugggcggc

SEQ ID NO: 66 - RNA, 1237 nt, Artificial Sequence
  source: /note="Description of Artificial Sequence: Synthetic polynucleotide"
gggaaauaagagagaaaagaagaguaagaagaaauauaagagccaccauggaggagggcaugaacgugcuucacgacuucggcauccagucaacccauuaccuacaggugaacuaucaggacucccaggauugguucauccucgugagcgugaucgccgaucuaagaaacgcauucuacguguuguucccaaucugguuccaccugcaggaagcugugggcaucaagcuccuuuggguggccgugauuggcgauuggcugaaccugguguucaaguggauucucuucggucagcggccuuacugguggguguuggauaccgacuauuacaguaacaccucuguuccgcugaucaagcaguucccugucaccugcgaaaccggaccuggcuccccuuccggccacgccaugggcaccgccggcguguacuacgugauggugacauccacccugagcaucuuccagggcaagaucaagccuaccuacagauucaggugccugaacguuaucuuguggcugggauucugggcagugcagcucaacgugugccugagcaggaucuaucucgcagcccacuucccacaucaggucguggccggcguacugagcggaaucgccguggcugaaaccuucagccauauccacagcaucuacaaugccucccugaagaaguacuuccuuauuacauucuuccuguucucuuucgccaucggcuucuaucugcugcuaaagggccugggcgucgaccuccuguggacccuggagaaggcccagagauggugcgaacaaccugagugggugcacaucgacaccacuccguucgcuagccugcucaagaaccugggcacucuuuucggccugggccuggcccucaauagcagcauguaccgggagagcuguaagggaaagcuguccaaguggcucccuuucagacuuagcugcaucguggcgucucucgugcugcugcacguguucgacagccugaagccuccuucgcagguggagcugguguucuacgugcugagcuucugcaagagcgcgguggugccacuggcaagugucagcgugaucccuuauugccuggcccaggugcugggccagccucauaagaagucccugugauaauaggcuggagccucgguggccuagcuucuugccccuugggccuccccccagccccuccuccccuuccugcacccguacccccguggucuuugaauaaagucugagugggcggc

SEQ ID NO: 67 - RNA, 1237 nt, Artificial Sequence
  source: /note="Description of Artificial Sequence: Synthetic polynucleotide"
gggaaauaagagagaaaagaagaguaagaagaaauauaagagccaccauggaggagggcaugaacgugcuucacgacuucggcauccagucaacccauuaccuacaggugaacuaucaggacucccaggauugguucauccucgugagcgugaucgccgaucuaagaaacgcauucuacguguuguucccaaucugguuccaccugcaggaagcugugggcaucaagcuccuuuggguggccgugauuggcgauuggcugaaccugguguucaaguggauucucuucggucagcggccuuacugguggguguuggauaccgacuauuacaguaacaccucuguuccgcugaucaagcaguucccugucaccugcgaaaccggaccuggcuccccuuccggccacgccaugggcaccgccggcguguacuacgugauggugacauccacccugagcaucuucaggggcaagaucaagccuaccuacagauucaggugccugaacguuaucuuguggcugggauucugggcagugcagcucaacgugugccugagcaggaucuaucucgcagcccacuucccacaucaggucguggccggcguacugagcggaaucgccguggcugaaaccuucagccauauccacagcaucuacaaugccucccugaagaaguacuuccuuauuacauucuuccuguucucuuucgccaucggcuucuaucugcugcuaaagggccugggcgucgaccuccuguggacccuggagaaggcccagagauggugcgaacggccugagugggugcacaucgacaccacuccguucgcuagccugcucaagaaccugggcacucuuuucggccugggccuggcccucaauagcagcauguaccgggagagcuguaagggaaagcuguccaaguggcucccuuucagacuuagcugcaucguggcgucucucgugcugcugcacguguucgacagccugaagccuccuucgcagguggagcugguguucuacgugcugagcuucugcaagagcgcgguggugccacuggcaagugucagcgugaucccuuauugccuggcccaggugcugggccagccucauaagaagucccugugauaauaggcuggagccucgguggccuagcuucuugccccuugggccuccccccagccccuccuccccuuccugcacccguacccccguggucuuugaauaaagucugagugggcggc

SEQ ID NO: 68 - RNA, 1237 nt, Artificial Sequence
  source: /note="Description of Artificial Sequence: Synthetic polynucleotide"
gggaaauaagagagaaaagaagaguaagaagaaauauaagagccaccauggaggagggcaugaacgugcuucacgacuucggcauccagucaacccauuaccuacaggugaacuaucaggacucccaggauugguucauccucgugagcgugaucgccgaucuaagaaacgcauucuacguguuguucccaaucugguuccaccugcaggaagcugugggcaucaagcuccuuuggguggccgugauuggcgauuggcugaaccugguguucaaguggauucucuucggucagcggccuuacugguggguguuggauaccgacuauuacaguaacaccucuguuccgcugaucaagcaguucccugucaccugcgaaaccggaccuggcuccccuuccggccacgccaugggcaccgccggcguguacuacgugauggugacauccacccugagcaucuucaggggcaagaagaagccuaccuacagauucaggugccugaacguuaucuuguggcugggauucugggcagugcagcucaacgugugccugagcaggaucuaucucgcagcccacuucccacaucaggucguggccggcguacugagcggaaucgccguggcugaaaccuucagccauauccacagcaucuacaaugccucccugaagaaguacuuccuuauuacauucuuccuguucucuuucgccaucggcuucuaucugcugcuaaagggccugggcgucgaccuccuguggacccuggagaaggcccagagauggugcgaacggccugagugggugcacaucgacaccacuccguucgcuagccugcucaagaaccugggcacucuuuucggccugggccuggcccucaauagcagcauguaccgggagagcuguaagggaaagcuguccaaguggcucccuuucagacuuggaugcaucguggcgucucucgugcugcugcaccuguucgacagccugaagccuccuucgcagguggagcugauuuucuacgugcugagcuucugcaagagcgcgguggugccacuggcaagugucagccugaucccuuauugccuggcccaggugcugggccagccucauaagaagucccugugauaauaggcuggagccucgguggccuagcuucuugccccuugggccuccccccagccccuccuccccuuccugcacccguacccccguggucuuugaauaaagucugagugggcggc

SEQ ID NO: 69 - RNA, 1237 nt, Artificial Sequence
  source: /note="Description of Artificial Sequence: Synthetic polynucleotide"
gggaaauaagagagaaaagaagaguaagaagaaauauaagagccaccauggaggagggcaugaacguacuucacgacuucggcauccagagcacccacuacuugcaggugaacuaccaggacucccaggauugguucauucucgugagcgugauugccgaucuccggaacgcuuucuacgugcuguucccuauuugguuccaccugcaggaggcugugggcaucaaguugcugugggucgccgugauaggcgacuggcucaacuugguguucaaguggauucuguucggccagcguccauacuggugggugcuggacacagacuauuauucuaauacaagcguaccucugaucaagcaguucccagugaccugcgaaacgggaccuggaucaccaagcggccacgccaugggaacggcuggcguguacuacgugauggugaccagcacccucagcaucuuccagggaaagaucaagccgacuuacagauuccguugccugaacgugauccuguggcucggauucugggccgugcagcucaacgugugccugaguagaaucuaccuggccgcucacuucccucaccagguaguggccggcgugcugagcggcauugccguggccgagacauucagucacauccacagcaucuauaacgcuagccugaagaaguauuuccugauuacauucuuccuguucucuuucgcuaucggcuucuaccuccuccugaagggccugggcguggaccuguuguggacccuggagaaggcucagagguggugcgagcaaccugaguggguccauaucgauaccaccccauucgcaagucugcugaagaaccugggcacacucuucggccugggccuggcccugaacagcucgauguacagagagucuugcaagggaaagcuuagcaaguggcucccuuucagacugucuugcaucguggccagccuggugcugcugcauguguucgacucucugaagccuccuucacaggucgagcugguuuucuaugugcugaguuucugcaaguccgcuguggugccucuggcuagcgugagcgugaucccuuacugccuggcccaggugcugggccagccucacaagaagucccuaugauaauaggcuggagccucgguggccuagcuucuugccccuugggccuccccccagccccuccuccccuuccugcacccguacccccguggucuuugaauaaagucugagugggcggc

SEQ ID NO: 70 - RNA, 1237 nt, Artificial Sequence
  source: /note="Description of Artificial Sequence: Synthetic polynucleotide"
gggaaauaagagagaaaagaagaguaagaagaaauauaagagccaccauggaggagggcaugaacguacuucacgacuucggcauccagagcacccacuacuugcaggugaacuaccaggacucccaggauugguucauucucgugagcgugauugccgaucuccggaacgcuuucuacgugcuguucccuauuugguuccaccugcaggaggcugugggcaucaaguugcugugggucgccgugauaggcgacuggcucaacuugguguucaaguggauucuguucggccagcguccauacuggugggugcuggacacagacuauuauucuaauacaagcguaccucugaucaagcaguucccagugaccugcgaaacgggaccuggaucaccaagcggccacgccaugggaacggcuggcguguacuacgugauggugaccagcacccucagcaucuuccggggaaagaucaagccgacuuacagauuccguugccugaacgugauccuguggcucggauucugggccgugcagcucaacgugugccugaguagaaucuaccuggccgcucacuucccucaccagguaguggccggcgugcugagcggcauugccguggccgagacauucagucacauccacagcaucuauaacgcuagccugaagaaguauuuccugauuacauucuuccuguucucuuucgcuaucggcuucuaccuccuccugaagggccugggcguggaccuguuguggacccuggagaaggcucagagguggugcgagaggccugaguggguccauaucgauaccaccccauucgcaagucugcugaagaaccugggcacacucuucggccugggccuggcccugaacagcucgauguacagagagucuugcaagggaaagcuuagcaaguggcucccuuucagacugucuugcaucguggccagccuggugcugcugcauguguucgacucucugaagccuccuucacaggucgagcugguuuucuaugugcugaguuucugcaaguccgcuguggugccucuggcuagcgugagcgugaucccuuacugccuggcccaggugcugggccagccucacaagaagucccuaugauaauaggcuggagccucgguggccuagcuucuugccccuugggccuccccccagccccuccuccccuuccugcacccguacccccguggucuuugaauaaagucugagugggcggc

SEQ ID NO: 71 - RNA, 1237 nt, Artificial Sequence
  source: /note="Description of Artificial Sequence: Synthetic polynucleotide"
gggaaauaagagagaaaagaagaguaagaagaaauauaagagccaccauggaggagggcaugaacguacuucacgacuucggcauccagagcacccacuacuugcaggugaacuaccaggacucccaggauugguucauucucgugagcgugauugccgaucuccggaacgcuuucuacgugcuguucccuauuugguuccaccugcaggaggcugugggcaucaaguugcugugggucgccgugauaggcgacuggcucaacuugguguucaaguggauucuguucggccagcguccauacuggugggugcuggacacagacuauuauucuaauacaagcguaccucugaucaagcaguucccagugaccugcgaaacgggaccuggaucaccaagcggccacgccaugggaacggcuggcguguacuacgugauggugaccagcacccucagcaucuuccggggaaagaagaagccgacuuacagauuccguugccugaacgugauccuguggcucggauucugggccgugcagcucaacgugugccugaguagaaucuaccuggccgcucacuucccucaccagguaguggccggcgugcugagcggcauugccguggccgagacauucagucacauccacagcaucuauaacgcuagccugaagaaguauuuccugauuacauucuuccuguucucuuucgcuaucggcuucuaccuccuccugaagggccugggcguggaccuguuguggacccuggagaaggcucagagguggugcgagaggccugaguggguccauaucgauaccaccccauucgcaagucugcugaagaaccugggcacacucuucggccugggccuggcccugaacagcucgauguacagagagucuugcaagggaaagcuuagcaaguggcucccuuucagacugggaugcaucguggccagccuggugcugcugcaucuguucgacucucugaagccuccuucacaggucgagcugauuuucuaugugcugaguuucugcaaguccgcuguggugccucuggcuagcgugagccugaucccuuacugccuggcccaggugcugggccagccucacaagaagucccuaugauaauaggcuggagccucgguggccuagcuucuugccccuugggccuccccccagccccuccuccccuuccugcacccguacccccguggucuuugaauaaagucugagugggcggc

SEQ ID NO: 72 - RNA, 1237 nt, Artificial Sequence
  source: /note="Description of Artificial Sequence: Synthetic polynucleotide"
gggaaauaagagagaaaagaagaguaagaagaaauauaagagccaccauggaggaaggaaugaacgugcuucacgauuucggcauucaaagcacccauuaccuccaggugaacuaccaggacagccaggacugguucauuuuggucagcguaauugccgaucucaggaacgcauucuacgugcuguucccuaucugguuccaccugcaggaagccgugggcauuaagcugcuuuggguggccgugaucggcgacuggcugaaccugguguucaaguggauccuguucggccagcggccauacuggugggugcuggauaccgacuacuacagcaacacuucugucccgcugauaaagcaguucccgguaacgugcgaaacgggcccuggcagcccuagcggacacgccaugggcaccgccggcguguacuacgugauggugacuucgacccucagcauuuuccagggaaagaucaagccaaccuacagauucaggugucucaaugugauucuguggcugggcuucugggcugugcaguugaacgugugccucagcagaauuuaccuggccgcccacuucccucaccaggugguggccggugugcugagcggcauugcuguggccgagacguucucgcauauccacagcaucuacaacgccagcuuaaagaaguacuuccugaucaccuucuuccucuucuccuucgcuaucggauucuaucugcugcugaagggacugggcgucgaccugcuguggacgcuggagaaggcccagcgguggugcgagcagccagagugggugcauaucgauacuaccccauucgccucucuguuaaagaaccugggcacacuguucggucugggccuggcccucaacuccagcauguaccgggagagcugcaagggaaagcuguccaaguggcugccuuuccgccugggcugcaucguggcuagccuuguccugcugcaucucuucgacagccucaagccuccaagccagguggaacugauuuucuacgugcugagcuucugcaagucagcuguggugccacuggcuagcgugucacugauuccuuacugccucgcccaggucuuaggccagccucauaagaagucgcugugauaauaggcuggagccucgguggccaugcuucuugccccuugggccuccccccagccccuccuccccuuccugcacccguacccccguggucuuugaauaaagucugagugggcggc

SEQ ID NO: 73 - RNA, 1237 nt, Artificial Sequence
  source: /note="Description of Artificial Sequence: Synthetic polynucleotide"
gggaaauaagagagaaaagaagaguaagaagaaauauaagagccaccauggaggagggaaugaacgucuuacacgacuucggcauccaguccacccacuaccuacaggugaauuaccaggacagccaagauugguucauccucgugagcguuauagccgacuugagaaacgccuucuacguguuguucccaaucugguuccaccuccaggaggcaguuggaauuaagcugcuguggguggcagugaucggcgacuggcugaaccuggucuucaaguggauuuuguucggccagaggccuuacuggugggugcuggauacagacuacuacuccaacacaagcgugccgcugauuaagcaguucccugugaccugugagacaggcccuggcuccccaagcggccacgccaugggcacagccgguguguacuacguuauggugacuagcacgcugucgauuuuccagggcaagaucaagccaaccuacagauucaggugccugaaugugauccuguggcucggcuucugggccguccagcugaacgugugccugagccgcaucuaucuggcggcucacuucccacaccaagugguugccggagugcucagcggcaucgcagucgccgaaaccuucagccacauucacagcauuuauaaugcuagccugaagaaguauuuccugaucaccuucuuccucuucagcuucgccauuggcuucuaucugcugcucaagggccugggcguggaccuucuguggacacuggagaaggcucagcgcuggugcgaacagccagagugggugcacaucgacaccaccccguucgccucccugcugaagaaucugggcacccuguucggccucggccuggcccugaacaguagcauguacagggaaagcuguaagggcaagcugagcaaguggcucccauuccggcugggcugcaucguugccagccuggugcugcugcaccuuuucgacucccugaagccaccuucacagguggagcucaucuucuacgugcucuccuucugcaaguccgcuguggugccgcuggcgagugugagccugaucccauacugccuugcccaggugcugggucagccucauaagaaguccuugugauaauaggcuggagccucgguggccaugcuucuugccccuugggccuccccccagccccuccuccccuuccugcacccguacccccguggucuuugaauaaagucugagugggcggc

SEQ ID NO: 74 - RNA, 1237 nt, Artificial Sequence
  source: /note="Description of Artificial Sequence: Synthetic polynucleotide"
gggaaauaagagagaaaagaagaguaagaagaaauauaagagccaccauggaggagggcaugaacgugcuucacgacuucggcauccagucaacccauuaccuacaggugaacuaucaggacucccaggauugguucauccucgugagcgugaucgccgaucuaagaaacgcauucuacguguuguucccaaucugguuccaccugcaggaagcugugggcaucaagcuccuuuggguggccgugauuggcgauuggcugaaccugguguucaaguggauucucuucggucagcggccuuacugguggguguuggauaccgacuauuacaguaacaccucuguuccgcugaucaagcaguucccugucaccugcgaaaccggaccuggcuccccuuccggccacgccaugggcaccgccggcguguacuacgugauggugacauccacccugagcaucuuccagggcaagaucaagccuaccuacagauucaggugccugaacguuaucuuguggcugggauucugggcagugcagcucaacgugugccugagcaggaucuaucucgcagcccacuucccacaucaggucguggccggcguacugagcggaaucgccguggcugaaaccuucagccauauccacagcaucuacaaugccucccugaagaaguacuuccuuauuacauucuuccuguucucuuucgccaucggcuucuaucugcugcuaaagggccugggcgucgaccuccuguggacccuggagaaggcccagagauggugcgaacaaccugagugggugcacaucgacaccacuccguucgcuagccugcucaagaaccugggcacucuuuucggccugggccuggcccucaauagcagcauguaccgggagagcuguaagggaaagcuguccaaguggcucccuuucagacuuggaugcaucguggcgucucucgugcugcugcaccuguucgacagccugaagccuccuucgcagguggagcugauuuucuacgugcugagcuucugcaagagcgcgguggugccacuggcaagugucagccugaucccuuauugccuggcccaggugcugggccagccucauaagaagucccugugauaauaggcuggagccucgguggccaugcuucuugccccuugggccuccccccagccccuccuccccuuccugcacccguacccccguggucuuugaauaaagucugagugggcggc

SEQ ID NO: 75 - RNA, 1237 nt, Artificial Sequence
  source: /note="Description of Artificial Sequence: Synthetic polynucleotide"
gggaaauaagagagaaaagaagaguaagaagaaauauaagagccaccauggaggagggcaugaacgugcuccacgacuucggcauccagagcacccacuaccuccaggugaacuaccaggacagccaggacugguucauccucgugagcgugaucgccgacuugcggaacgccuucuacguguuguuccccaucugguuccacuugcaggaggccgugggcaucaagcugcuguggguggccgugaucggcgacuggcugaaccugguguucaaguggauccuguucggccagcggcccuacuggugggugcuggacaccgacuacuacagcaacaccagcgugccccugaucaagcaguuccccgugaccugcgagacgggccccggcagcccuucuggucacgccaugggcaccgccggcguguacuacgugauggugaccagcacccugagcaucuuccagggcaagaucaagcccaccuaccgguuccggugccugaacgugauccuguggcugggcuucugggccgugcagcugaaugugugccugagccggaucuaccuggccgcccacuucccacaccaggugguggccggcguccugagcggcaucgccguggccgagacguucagccacauccacagcaucuacaacgccagccugaagaaguacuuccugaucaccuucuuccuguucagcuucgccaucggcuucuaccugcugcugaagggccugggcguggaccuucuguggacccuggagaaggcccagcgguggugcgagcagcccgagugggugcacaucgacaccaccccauucgcaagccugcuaaagaaccugggcacacucuucggccugggacuggcccugaacagcagcauguaccgggagagcugcaagggcaagcugagcaaguggcugcccuucaggcuuggcugcaucguggcuagccuggugcugcugcaccuguucgacucccugaagccucccagccagguggagcugaucuucuauguccucagcuucugcaagagcgccguggugccacucgccagcgugagccugauccccuacugccuggcccaggugcugggccagccccacaagaagucccugugauaauaggcuggagccucgguggccaugcuucuugccccuugggccuccccccagccccuccuccccuuccugcacccguacccccguggucuuugaauaaagucugagugggcggc

SEQ ID NO: 76 - RNA, 1237 nt, Artificial Sequence
  source: /note="Description of Artificial Sequence: Synthetic polynucleotide"
gggaaauaagagagaaaagaagaguaagaagaaauauaagagccaccauggaggagggcaugaacgugcuccacgacuucggcauccagagcacccacuaccuccaggugaacuaccaggacagccaggacugguucaucuuggugagcgugaucgccgacuugcggaacgccuucuacgugcuguuccccaucugguuccaccugcaagaggccgugggcaucaagcugcuguggguggccgugaucggcgacuggcugaaccugguguucaaguggauccuguucggccagcggcccuacuggugggugcuggacaccgacuacuacagcaacaccagcgugccccugaucaagcaguuccccgugaccugcgagacuggccccggcagcccuagcggacacgccaugggcaccgccggcguguacuacgugauggugaccagcacccugagcaucuuccagggcaagaucaagcccaccuaccgguuccggugccugaacgugauccuguggcugggcuucugggccgugcagcucaaugucugccugagccggaucuaccuggccgcccacuucccucaccaggugguggccggaguucugagcggcaucgccguggccgagacuuucagccacauccacagcaucuacaacgccagccugaagaaguacuuccugaucaccuucuuccuguucagcuucgccaucggcuucuaccugcugcugaagggccugggcguggaccuucuguggacccuggagaaggcccagcgguggugcgagcagcccgagugggugcacaucgacaccacaccuuucgccucacugcucaagaaccugggcacgcuguucggacugggccuggcccugaacagcagcauguaccgggagagcugcaagggcaagcugagcaaguggcugcccuucagacugggaugcaucguggcgagcuuggugcugcugcaccuguucgauucccugaagccacccagccagguggagcugaucuucuauguccucagcuucuguaagagcgccguggugccgcuggccagcgugagccugauccccuacugucuggcccaggugcugggccagccccacaagaagucccugugauaauaggcuggagccucgguggccaugcuucuugccccuugggccuccccccagccccuccuccccuuccugcacccguacccccguggucuuugaauaaagucugagugggcggc

SEQ ID NO: 77 - RNA, 1237 nt, Artificial Sequence
  source: /note="Description of Artificial Sequence: Synthetic polynucleotide"
gggaaauaagagagaaaagaagaguaagaagaaauauaagagccaccauggaggagggcaugaacguacuucacgacuucggcauccagagcacccacuacuugcaggugaacuaccaggacucccaggauugguucauucucgugagcgugauugccgaucuccggaacgcuuucuacgugcuguucccuauuugguuccaccugcaggaggcugugggcaucaaguugcugugggucgccgugauaggcgacuggcucaacuugguguucaaguggauucuguucggccagcguccauacuggugggugcuggacacagacuauuauucuaauacaagcguaccucugaucaagcaguucccagugaccugcgaaacgggaccuggaucaccaagcggccacgccaugggaacggcuggcguguacuacgugauggugaccagcacccucagcaucuuccggggaaagaagaagccgacuuacagauuccguugccugaacgugauccuguggcucggauucugggccgugcagcucaacgugugccugaguagaaucuaccuggccgcucacuucccucaccagguaguggccggcgugcugagcggcauugccguggccgagacauucagucacauccacagcaucuauaacgcuagccugaagaaguauuuccugauuacauucuuccuguucucuuucgcuaucggcuucuaccuccuccugaagggccugggcguggaccuguuguggacccuggagaaggcucagagguggugcgagaggccugaguggguccauaucgauaccaccccauucgcaagucugcugaagaaccugggcacacucuucggccugggccuggcccugaacagcucgauguacagagagucuugcaagggaaagcuuagcaaguggcucccuuucagacugucuugcaucguggccagccuggugcugcugcaucuguucgacucucugaagccuccuucacaggucgagcugguuuucuaugugcugaguuucugcaaguccgcuguggugccucuggcuagcgugagcgugaucccuuacugccuggcccaggugcugggccagccucacaagaagucccuaugauaauaggcuggagccucgguggccaugcuucuugccccuugggccuccccccagccccuccuccccuuccugcacccguacccccguggucuuugaauaaagucugagugggcggc

SEQ ID NO: 78 - RNA, 1237 nt, Artificial Sequence
  source: /note="Description of Artificial Sequence: Synthetic polynucleotide"
gggaaauaagagagaaaagaagaguaagaagaaauauaagagccaccauggaggagggcaugaacguccuucacgacuucgguauccagucgacccacuaccuccaagugaacuaucaggauagccaggacugguucauuuuggugagcguaauagccgaccucagaaacgccuucuacguguuauucccuaucugguuccaccugcaggaggccgugggaauaaagcuucuuuggguggcugugauuggcgauuggcugaaccugguguucaaguggauccuguucggccagaggccauacugguggguccuggauaccgacuacuacagcaacacaagcgugccacugauuaagcaguucccggugacaugcgaaacaggcccuggcuccccuagcggccaugcuaugggcaccgccggcguguauuacgugauggugaccagcaccuugucuaucuuccgaggcaagaagaagccuaccuacagauucaggugccugaacgugauccucuggcugggcuucugggccgugcagcuaaacguuugccucuccagaaucuaccucgccgcccauuucccacaccaggugguggccggcguucugaguggcaucgccguggcugagacauucagccacauccauagcauuuacaacgccagcuugaagaaguauuuccugauuaccuucuuccuguucagcuucgccauaggcuucuaucuucuucugaagggccugggcguggaccugcuguggacccuggagaaggcccagcgguggugcgagaggccugaaugggugcauaucgauacaaccccuuucgccucccuacucaagaaccucggcacucuguucggccucggccucgcccugaacagcuccauguacagagagagcugcaagggcaagcucagcaaguggcugccauuccggcugagcugcauuguugccagccucgugcuccugcaccuguucgacagucucaagccuccuagucagguggagcugguguucuauguccugucauucugcaaguccgccguggugccucuggcuagcgugagcgucaucccauacugccuggcccaagugcugggacagccacacaagaagucguuaugauaauaggcuggagccucgguggccaugcuucuugccccuugggccuccccccagccccuccuccccuuccugcacccguacccccguggucuuugaauaaagucugagugggcggc

SEQ ID NO: 79 - RNA, 1237 nt, Artificial Sequence
  source: /note="Description of Artificial Sequence: Synthetic polynucleotide"
gggaaauaagagagaaaagaagaguaagaagaaauauaagagccaccauggaggaggguaugaacguccuacacgacuucggcauacagucuacccacuaucuucagguuaacuaccaggacagccaggacugguucauccuugugagcguuaucgccgaccuucgcaacgcguucuacgugcuuuucccuaucugguuccaccugcaggaggcuguaggcauuaagcugcugugggucgccgugaucggcgacuggcugaaucugguguucaaguggauccuguucggccaacgcccuuauugguggguccuggacacagauuacuauucaaauaccagcgugccauugauuaagcaguucccuguuaccugcgaaaccggcccuggcuccccuuccggccaugcaaugggaaccgccggcguguacuaugucauggugaccagcacccuuucaauuuuccggggcaagaagaagccuacuuacagguucagaugccugaacgugauccuguggcugggcuucugggccgugcagcucaacgugugccugagcagaaucuaucucgccgcucacuucccucaucagguggucgccggagugcucucaggcaucgccguggcggagacguucucccacauacacagcauuuacaacgcaagccugaagaaguacuuccugaucaccuucuuccuguucagcuucgccaucggauucuaccugcugcugaagggccucggcguugaccugcuguggacccuggagaaggcccagagauggugugagcguccugagugggugcacauugacaccacuccguucgcuagccugcugaagaaccugggcacccuguucggccugggacuggcucugaacagcagcauguauagggaguccugcaagggcaagcuaucaaaguggcugccuuuccggcugagcugcauuguggccagccuggugcugcugcaccuguucgacucccugaagccgccuucccagguggagcuggucuucuacgugcuuagcuucuguaagagcgccguggugccacucgcuagcgugucuguuaucccuuacugccuggcccaggugcugggccagccucauaagaagucucucugauaauaggcuggagccucgguggccaugcuucuugccccuugggccuccccccagccccuccuccccuuccugcacccguacccccguggucuuugaauaaagucugagugggcggc

SEQ ID NO: 80 - RNA, 1237 nt, Artificial Sequence
  source: /note="Description of Artificial Sequence: Synthetic polynucleotide"
gggaaauaagagagaaaagaagaguaagaagaaauauaagagccaccauggaggagggcaugaacgugcuucacgauuucggaauucagagcacccacuacuugcaggugaacuaccaggacucucaagacugguucauccuugugagcgugaucgccgaucucaggaacgccuucuacguguuguucccgauuugguuccaccuucaggaggccgucggcaucaagcugcuguggguggccgugaucggcgacuggcugaacuugguguucaaguggauucuguucggacagaggccauacuggugggugcuggacacugacuauuauaguaacacuagcgucccacugauaaagcaauucccugugaccugcgagacaggcccuggcagcccuuccggccacgccaugggcacugccggaguauacuaugugauggugaccagcacccugagcaucuucaggggaaagaagaagccuacguacagauucagaugccugaacgugauccuguggcugggcuucugggccgugcaacugaaugugugccucuccaggauuuaccuggcagcgcacuucccucaccaggucguggcuggagugcugucuggaaucgccguggccgaaacauucagccacauucacucaauuuacaaugccagccugaagaaguacuuccugaucaccuucuuccuguucaguuucgccauagguuucuaccugcugcucaagggccuaggcguugaccugcuguggacauuggagaaggcacagcgcuggugcgagaggccagaaugggugcacauugacacaaccccuuucgccagccuccugaagaaucucggcacccuguucggccugggccuggcccugaacagcucaauguauagagagagcugcaaggguaagcugagcaaguggcugccuuucaggcugagcugcaucguugccagccucguacugcuccaccucuucgacucucugaagccaccaagucagguggagcugguguucuaugugcuuagcuucugcaagagcgccguggugccucuggccagcguguccgugaucccuuacugccuggcccagguccugggccagccgcauaagaagucucugugauaauaggcuggagccucgguggccaugcuucuugccccuugggccuccccccagccccuccuccccuuccugcacccguacccccguggucuuugaauaaagucugagugggcggc

SEQ ID NO: 81 - RNA, 1237 nt, Artificial Sequence
  source: /note="Description of Artificial Sequence: Synthetic polynucleotide"
gggaaauaagagagaaaagaagaguaagaagaaauauaagagccaccauggaggagggcaugaacguguuacacgacuucggcauccagagcacccacuaccuccaggugaacuaccaggacagccaggacugguucauccuagugagcgugaucgccgacuuacggaacgccuucuacgugcuuuuccccaucugguuccaccuucaggaggccgugggcaucaagcugcuguggguggccgugaucggcgacuggcugaaccugguguucaaguggauccuguucggccagcggcccuacuggugggugcuggacaccgacuacuacagcaacaccagcgugccccugaucaagcaguuccccgugaccugcgagacaggccccggcagcccgagcggccacgccaugggcaccgccggcguguacuacgugauggugaccagcacccugagcaucuuccggggcaagaagaagcccaccuaccgguuccggugccugaacgugauccuguggcugggcuucugggccgugcagcuuaacgucugccugagccggaucuaccuggccgcccacuucccucaccaggugguggcuggagugcugagcggcaucgccguggccgagacauucagccacauccacagcaucuacaacgccagccugaagaaguacuuccugaucaccuucuuccuguucagcuucgccaucggcuucuaccugcugcugaagggccugggcguggaccugcucuggacccuggagaaggcccagcgguggugcgaaagacccgagugggugcacaucgacaccaccccuuucgccucucugcucaagaaccugggcacgcuuuucggucugggccuggcccugaacagcagcauguaccgggagagcugcaagggcaagcugagcaaguggcugcccuuccggcugagcugcaucguggcuagccuggugcugcugcaccuguucgauucccugaagccucccagccagguggagcucguguucuaugugcugucauucugcaagagcgccguggugccacuggccagcgugucagugauccccuacugucuggcacaggugcugggccagccccacaagaagucucugugauaauaggcuggagccucgguggccaugcuucuugccccuugggccuccccccagccccuccuccccuuccugcacccguacccccguggucuuugaauaaagucugagugggcggc

SEQ ID NO: 82 - protein, 365 aa, Artificial Sequence
  source: /note="Description of Artificial Sequence: Synthetic polypeptide"
MEEGMNILHDFGIQSTRYLQVNYQDSQDWFILVSVIADLRNAFYVLFPIWFHLKETVGINLLWVAVVGDWFNLVFKWILFGQRPYWWVLDTDYYSNSSVPIIKQFPVTCETGPGSPSGHAMGAAGVYYVMVTSTLAIFRGKKKPTYGFRCLNVILWLGFWAVQLNVCLSRIYLAAHFPHQVVAGVLSGIAVAETFSHIRGIYNASLRKYCLITIFLFGFALGFYLLLKGLGVDLLWTLEKAKRWCERPEWVHLDTTPFASLFKNLGTLLGLGLALNSSMYRKSCKGELSKLLPFRFACIVASLVLLHLFDSLKPPSQVELIFYILSFCKSATVPFASVSLIPYCLARILGQTHKKSLDYKDDDDK

SEQ ID NO: 83 - protein, 357 aa, Artificial Sequence
  source: /note="Description of Artificial Sequence: Synthetic polypeptide"
MEEGMNVLHDFGIQSTHYLQVNYQDSQDWFILVSVIADLRNAFYVLFPIWFHLQEAVGIKLLWVAVIGDWLNLVFKWILFGQRPYWWVLDTDYYSNTSVPLIKQFPVTCETGPGSPSGHAMGTAGVYYVMVTSTLSIFQGKIKPTYRFRCLNVILWLGFWAVQLNVCLSRIYLAAHFPHQVVAGVLSGIAVAETFSHIHSIYNASLKKYFLITFFLFSFAIGFYLLLKGLGVDLLWTLEKAQRWCEQPEWVHIDTTPFASLLKNLGTLFGLGLALNSSMYRESCKGKLSKWLPFRLGCIVASLVLLHLFDSLKPPSQVELIFYVLSFCKSAVVPLASVSLIPYCLAQVLGQPHKKSL

SEQ ID NO: 84 - protein, 357 aa, Artificial Sequence
  source: /note="Description of Artificial Sequence: Synthetic polypeptide"
MEEGMNVLHDFGIQSTHYLQVNYQDSQDWFILVSVIADLRNAFYVLFPIWFHLQEAVGIKLLWVAVIGDWLNLVFKWILFGQRPYWWVLDTDYYSNTSVPLIKQFPVTCETGPGSPSGHAMGTAGVYYVMVTSTLSIFRGKKKPTYRFRCLNVILWLGFWAVQLNVCLSRIYLAAHFPHQVVAGVLSGIAVAETFSHIHSIYNASLKKYFLITFFLFSFAIGFYLLLKGLGVDLLWTLEKAQRWCERPEWVHIDTTPFASLLKNLGTLFGLGLALNSSMYRESCKGKLSKWLPFRLSCIVASLVLLHLFDSLKPPSQVELVFYVLSFCKSAVVPLASVSVIPYCLAQVLGQPHKKSL

SEQ ID NO: 85 - RNA, 41 nt, Artificial Sequence
  source: /note="Description of Artificial Sequence: Synthetic oligonucleotide"
gggaaauaagagagaaaagaagaguaagaagaaauauaaga

SEQ ID NO: 86 - protein, 5 aa, Artificial Sequence
  source: /note="Description of Artificial Sequence: Synthetic peptide"
GGGGS

SEQ ID NO: 87 - RNA, 9 nt, Artificial Sequence
  source: /note="Description of Artificial Sequence: Synthetic oligonucleotide"
ccrccaugg

SEQ ID NO: 88 - RNA, 92 nt, Artificial Sequence
  source: /note="Description of Artificial Sequence: Synthetic oligonucleotide"
ucaagcuuuuggacccucguacagaagcuaauacgacucacuauagggaaauaagagagaaaagaagaguaagaagaaauauaagagccacc

SEQ ID NO: 89 - RNA, 47 nt, Artificial Sequence
  source: /note="Description of Artificial Sequence: Synthetic oligonucleotide"
gggagaucagagagaaaagaagaguaagaagaaauauaagagccacc

SEQ ID NO: 90 - RNA, 42 nt, Artificial Sequence
  source: /note="Description of Artificial Sequence: Synthetic oligonucleotide"
gggagacaagcuuggcauuccgguacuguugguaaagccacc

SEQ ID NO: 91 - RNA, 47 nt, Artificial Sequence; identical to SEQ ID NO: 89
  source: /note="Description of Artificial Sequence: Synthetic oligonucleotide"

SEQ ID NO: 92 - RNA, 42 nt, Artificial Sequence; identical to SEQ ID NO: 90
  source: /note="Description of Artificial Sequence: Synthetic oligonucleotide"

SEQ ID NO: 93 - RNA, 47 nt, Artificial Sequence
  source: /note="Description of Artificial Sequence: Synthetic oligonucleotide"
gggaauuaacagagaaaagaagaguaagaagaaauauaagagccacc

SEQ ID NO: 94 - RNA, 47 nt, Artificial Sequence
  source: /note="Description of Artificial Sequence: Synthetic oligonucleotide"
gggaaauuagacagaaaagaagaguaagaagaaauauaagagccacc

SEQ ID NO: 95 - RNA, 47 nt, Artificial Sequence
  source: /note="Description of Artificial Sequence: Synthetic oligonucleotide"
gggaaauaagagaguaaagaacaguaagaagaaauauaagagccacc

SEQ ID NO: 96 - RNA, 47 nt, Artificial Sequence
  source: /note="Description of Artificial Sequence: Synthetic oligonucleotide"
gggaaaaaagagagaaaagaagacuaagaagaaauauaagagccacc

SEQ ID NO: 97 - RNA, 47 nt, Artificial Sequence
  source: /note="Description of Artificial Sequence: Synthetic oligonucleotide"
gggaaauaagagagaaaagaagaguaagaagauauauaagagccacc

SEQ ID NO: 98 - RNA, 47 nt, Artificial Sequence
  source: /note="Description of Artificial Sequence: Synthetic oligonucleotide"
gggaaauaagagacaaaacaagaguaagaagaaauauaagagccacc

SEQ ID NO: 99 - RNA, 47 nt, Artificial Sequence
  source: /note="Description of Artificial Sequence: Synthetic oligonucleotide"
gggaaauuagagaguaaagaacaguaaguagaauuaaaagagccacc

SEQ ID NO: 100 - RNA, 47 nt, Artificial Sequence
  source: /note="Description of Artificial Sequence: Synthetic oligonucleotide"
gggaaauaagagagaauagaagaguaagaagaaauauaagagccacc

SEQ ID NO: 101 - RNA, 47 nt, Artificial Sequence
  source: /note="Description of Artificial Sequence: Synthetic oligonucleotide"
gggaaauaagagagaaaagaagaguaagaagaaaauuaagagccacc

SEQ ID NO: 102 - RNA, 47 nt, Artificial Sequence
  source: /note="Description of Artificial Sequence: Synthetic oligonucleotide"
gggaaauaagagagaaaagaagaguaagaagaaauuuaagagccacc

SEQ ID NO: 103 - skipped

SEQ ID NO: 104 - RNA, 142 nt, Artificial Sequence
  source: /note="Description of Artificial Sequence: Synthetic polynucleotide"
ugauaauaguccauaaaguaggaaacacuacagcuggagccucgguggccaugcuucuugccccuugggccuccccccagccccuccuccccuuccugcacccguacccccguggucuuugaauaaagucugagugggcggc

SEQ ID NO: 105 - RNA, 142 nt, Artificial Sequence
  source: /note="Description of Artificial Sequence: Synthetic polynucleotide"
ugauaauaggcuggagccucgguggcuccauaaaguaggaaacacuacacaugcuucuugccccuugggccuccccccagccccuccuccccuuccugcacccguacccccguggucuuugaauaaagucugagugggcggc

SEQ ID NO: 106 - RNA, 142 nt, Artificial Sequence
  source: /note="Description of Artificial Sequence: Synthetic polynucleotide"
ugauaauaggcuggagccucgguggccaugcuucuugccccuuccauaaaguaggaaacacuacaugggccuccccccagccccuccuccccuuccugcacccguacccccguggucuuugaauaaagucugagugggcggc

SEQ ID NO: 107 - RNA, 142 nt, Artificial Sequence
  source: /note="Description of Artificial Sequence: Synthetic polynucleotide"
ugauaauaggcuggagccucgguggccaugcuucuugccccuugggccuccccccaguccauaaaguaggaaacacuacaccccuccuccccuuccugcacccguacccccguggucuuugaauaaagucugagugggcggc

SEQ ID NO: 108 - RNA, 142 nt, Artificial Sequence
  source: /note="Description of Artificial Sequence: Synthetic polynucleotide"
ugauaauaggcuggagccucgguggccaugcuucuugccccuugggccuccccccagccccuccuccccuucuccauaaaguaggaaacacuacacugcacccguacccccguggucuuugaauaaagucugagugggcggc

SEQ ID NO: 109 - RNA, 142 nt, Artificial Sequence
  source: /note="Description of Artificial Sequence: Synthetic polynucleotide"
ugauaauaggcuggagccucgguggccaugcuucuugccccuugggccuccccccagccccuccuccccuuccugcacccguacccccuccauaaaguaggaaacacuacaguggucuuugaauaaagucugagugggcggc

SEQ ID NO: 110 - RNA, 142 nt, Artificial Sequence
  source: /note="Description of Artificial Sequence: Synthetic polynucleotide"
ugauaauaggcuggagccucgguggccaugcuucuugccccuugggccuccccccagccccuccuccccuuccugcacccguacccccguggucuuugaauaaaguuccauaaaguaggaaacacuacacugagugggcggc

SEQ ID NO: 111 - RNA, 164 nt, Artificial Sequence
  source: /note="Description of Artificial Sequence: Synthetic polynucleotide"
ugauaauaguccauaaaguaggaaacacuacagcuggagccucgguggccaugcuucuugccccuugggccuccccccagccccuccuccccuuccugcacccguaccccccgcauuauuacucacgguacgaguggucuuugaauaaagucugagugggcggc

SEQ ID NO: 112 - RNA, 164 nt, Artificial Sequence
  source: /note="Description of Artificial Sequence: Synthetic polynucleotide"
ugauaauaguccauaaaguaggaaacacuacagcuggagccucgguggccuagcuucuugccccuugggccuccccccagccccuccuccccuuccugcacccguaccccccgcauuauuacucacgguacgaguggucuuugaauaaagucugagugggcggc

SEQ ID NO: 113 - skipped

SEQ ID NO: 114 - RNA, 87 nt, Artificial Sequence
  source: /note="Description of Artificial Sequence: Synthetic oligonucleotide"
gacagugcagucacccauaaaguagaaagcacuacuaacagcacuggaggguguaguguuuccuacuuuauggaugaguguacugug

SEQ ID NO: 115 - RNA, 23 nt, Artificial Sequence
  source: /note="Description of Artificial Sequence: Synthetic oligonucleotide"
uguaguguuuccuacuuuaugga

SEQ ID NO: 116 - RNA, 23 nt, Artificial Sequence
  source: /note="Description of Artificial Sequence: Synthetic oligonucleotide"
uccauaaaguaggaaacacuaca

SEQ ID NO: 117 - RNA, 21 nt, Artificial Sequence
  source: /note="Description of Artificial Sequence: Synthetic oligonucleotide"
cauaaaguagaaagcacuacu

SEQ ID NO: 118 - RNA, 21 nt, Artificial Sequence
  source: /note="Description of Artificial Sequence: Synthetic oligonucleotide"
aguagugcuuucuacuuuaug

SEQ ID NO: 119 - RNA, 85 nt, Artificial Sequence
  source: /note="Description of Artificial Sequence: Synthetic oligonucleotide"
cgcuggcgacgggacauuauuacuuuugguacgcgcugugacacuucaaacucguaccgugaguaauaaugcgccguccacggca

SEQ ID NO: 120 - RNA, 22 nt, Artificial Sequence
  source: /note="Description of Artificial Sequence: Synthetic oligonucleotide"
ucguaccgugaguaauaaugcg

SEQ ID NO: 121 - RNA, 22 nt, Artificial Sequence
  source: /note="Description of Artificial Sequence: Synthetic oligonucleotide"
cgcauuauuacucacgguacga

SEQ ID NO: 122 - RNA, 21 nt, Artificial Sequence
  source: /note="Description of Artificial Sequence: Synthetic oligonucleotide"
cauuauuacuuuugguacgcg

SEQ ID NO: 123 - RNA, 21 nt, Artificial Sequence
  source: /note="Description of Artificial Sequence: Synthetic oligonucleotide"
cgcguaccaaaaguaauaaug

SEQ ID NO: 124 - RNA, 9 nt, Artificial Sequence
  source: /note="Description of Artificial Sequence: Synthetic oligonucleotide"
ugauaauag

SEQ ID NO: 125 - RNA, 9 nt, Artificial Sequence
  source: /note="Description of Artificial Sequence: Synthetic oligonucleotide"
ugauaguaa

SEQ ID NO: 126 - RNA, 9 nt, Artificial Sequence
  source: /note="Description of Artificial Sequence: Synthetic oligonucleotide"
uaaugauag

SEQ ID NO: 127 - RNA, 9 nt, Artificial Sequence
  source: /note="Description of Artificial Sequence: Synthetic oligonucleotide"
ugauaauaa

SEQ ID NO: 128 - RNA, 9 nt, Artificial Sequence
  source: /note="Description of Artificial Sequence: Synthetic oligonucleotide"
ugauaguag

SEQ ID NO: 129 - RNA, 9 nt, Artificial Sequence
  source: /note="Description of Artificial Sequence: Synthetic oligonucleotide"
uaaugauga

SEQ ID NO: 130 - RNA, 9 nt, Artificial Sequence
  source: /note="Description of Artificial Sequence: Synthetic oligonucleotide"
uaauaguag

SEQ ID NO: 131 - RNA, 9 nt, Artificial Sequence
  source: /note="Description of Artificial Sequence: Synthetic oligonucleotide"
ugaugauga

SEQ ID NO: 132 - RNA, 9 nt, Artificial Sequence
  source: /note="Description of Artificial Sequence: Synthetic oligonucleotide"
uaauaauaa

SEQ ID NO: 133 - RNA, 9 nt, Artificial Sequence
  source: /note="Description of Artificial Sequence: Synthetic oligonucleotide"
uaguaguag

SEQ ID NO: 134 - RNA, 133 nt, Artificial Sequence
  source: /note="Description of Artificial Sequence: Synthetic polynucleotide"
gcuggagccucgguggccaugcuucuugccccuugggccuccccccagccccuccuccccuuccugcacccguacccccuccauaaaguaggaaacacuacaguggucuuugaauaaagucugagugggcggc

SEQ ID NO: 135 - RNA, 22 nt, Artificial Sequence
  source: /note="Description of Artificial Sequence: Synthetic oligonucleotide"
ccucugaaauucaguucuucag

SEQ ID NO: 136 - RNA, 22 nt, Artificial Sequence
  source: /note="Description of Artificial Sequence: Synthetic oligonucleotide"
ugagaacugaauuccauggguu

SEQ ID NO: 137 - RNA, 22 nt, Artificial Sequence
  source: /note="Description of Artificial Sequence: Synthetic oligonucleotide"
cuccuacauauuagcauuaaca

SEQ ID NO: 138 - RNA, 23 nt, Artificial Sequence
  source: /note="Description of Artificial Sequence: Synthetic oligonucleotide"
uuaaugcuaaucgugauaggggu

SEQ ID NO: 139 - RNA, 22 nt, Artificial Sequence
  source: /note="Description of Artificial Sequence: Synthetic oligonucleotide"
ccaguauuaacugugcugcuga

SEQ ID NO: 140 - RNA, 22 nt, Artificial Sequence
  source: /note="Description of Artificial Sequence: Synthetic oligonucleotide"
uagcagcacguaaauauuggcg

SEQ ID NO: 141 - RNA, 21 nt, Artificial Sequence
  source: /note="Description of Artificial Sequence: Synthetic oligonucleotide"
caacaccagucgaugggcugu

SEQ ID NO: 142 - RNA, 22 nt, Artificial Sequence
  source: /note="Description of Artificial Sequence: Synthetic oligonucleotide"
uagcuuaucagacugauguuga

SEQ ID NO: 143 - RNA, 22 nt, Artificial Sequence
  source: /note="Description of Artificial Sequence: Synthetic oligonucleotide"
ugucaguuugucaaauacccca

SEQ ID NO: 144 - RNA, 22 nt, Artificial Sequence
  source: /note="Description of Artificial Sequence: Synthetic oligonucleotide"
cguguauuugacaagcugaguu

SEQ ID NO: 145 - RNA, 22 nt, Artificial Sequence
  source: /note="Description of Artificial Sequence: Synthetic oligonucleotide"
uggcucaguucagcaggaacag

SEQ ID NO: 146 - RNA, 22 nt, Artificial Sequence
  source: /note="Description of Artificial Sequence: Synthetic oligonucleotide"
ugccuacugagcugauaucagu

SEQ ID NO: 147 - RNA, 21 nt, Artificial Sequence
  source: /note="Description of Artificial Sequence: Synthetic oligonucleotide"
uucacaguggcuaaguuccgc

SEQ ID NO: 148 - RNA, 22 nt, Artificial Sequence
  source: /note="Description of Artificial Sequence: Synthetic oligonucleotide"
agggcuuagcugcuugugagca

SEQ ID NO: 149 - RNA, 141 nt, Artificial Sequence
  source: /note="Description of Artificial Sequence: Synthetic polynucleotide"
ugauaauaggcuggagccucgguggccaugcuucuugccccuugggccuccccccagccccuccuccccuuccugcacccguaccccccgcauuauuacucacgguacgaguggucuuugaauaaagucugagugggcggc

SEQ ID NO: 150 - RNA, 119 nt, Artificial Sequence
  source: /note="Description of Artificial Sequence: Synthetic polynucleotide"
ugauaauaggcuggagccucgguggccaugcuucuugccccuugggccuccccccagccccuccuccccuuccugcacccguacccccguggucuuugaauaaagucugagugggcggc

SEQ ID NO: 151 - RNA, 142 nt, Artificial Sequence; identical to SEQ ID NO: 109
  source: /note="Description of Artificial Sequence: Synthetic polynucleotide"

SEQ ID NO: 152 - skipped

SEQ ID NO: 153 - RNA, 23 nt, Artificial Sequence
  source: /note="Description of Artificial Sequence: Synthetic oligonucleotide"
uuaaugcuaauugugauaggggu

SEQ ID NO: 154 - RNA, 23 nt, Artificial Sequence
  source: /note="Description of Artificial Sequence: Synthetic oligonucleotide"
accccuaucacaauuagcauuaa

SEQ ID NO: 155 - RNA, 188 nt, Artificial Sequence
  source: /note="Description of Artificial Sequence: Synthetic polynucleotide"
ugauaauaguccauaaaguaggaaacacuacagcuggagccucgguggccaugcuucuugccccuugggccuccauaaaguaggaaacacuacauccccccagccccuccuccccuuccugcacccguacccccuccauaaaguaggaaacacuacaguggucuuugaauaaagucugagugggcggc

SEQ ID NO: 156 - RNA, 140 nt, Artificial Sequence
  source: /note="Description of Artificial Sequence: Synthetic polynucleotide"
ugauaauaggcuggagccucgguggccaugcuucuugccccuugggccuccccccagccccuccuccccuuccugcacccguacccccaguagugcuuucuacuuuaugguggucuuugaauaaagucugagugggcggc

SEQ ID NO: 157 - RNA, 182 nt, Artificial Sequence
  source: /note="Description of Artificial Sequence: Synthetic polynucleotide"
ugauaauagaguagugcuuucuacuuuauggcuggagccucgguggccaugcuucuugccccuugggccaguagugcuuucuacuuuauguccccccagccccuccuccccuuccugcacccguacccccaguagugcuuucuacuuuaugguggucuuugaauaaagucugagugggcggc

SEQ ID NO: 158 - RNA, 184 nt, Artificial Sequence
  source: /note="Description of Artificial Sequence: Synthetic polynucleotide"
ugauaauagaguagugcuuucuacuuuauggcuggagccucgguggccaugcuucuugccccuugggccuccauaaaguaggaaacacuacauccccccagccccuccuccccuuccugcacccguacccccaguagugcuuucuacuuuaugguggucuuugaauaaagucugagugggcggc

SEQ ID NO: 159 - RNA, 142 nt, Artificial Sequence
  source: /note="Description of Artificial Sequence: Synthetic polynucleotide"
ugauaauaggcuggagccucgguggccaugcuucuugccccuugggccuccccccagccccuccuccccuuccugcacccguacccccaccccuaucacaauuagcauuaaguggucuuugaauaaagucugagugggcggc

SEQ ID NO: 160 - RNA, 188 nt, Artificial Sequence
  source: /note="Description of Artificial Sequence: Synthetic polynucleotide"
ugauaauagaccccuaucacaauuagcauuaagcuggagccucgguggccaugcuucuugccccuugggccaccccuaucacaauuagcauuaauccccccagccccuccuccccuuccugcacccguacccccaccccuaucacaauuagcauuaaguggucuuugaauaaagucugagugggcggc

SEQ ID NO: 161 - RNA, 188 nt, Artificial Sequence
  source: /note="Description of Artificial Sequence: Synthetic polynucleotide"
ugauaauagaccccuaucacaauuagcauuaagcuggagccucgguggccaugcuucuugccccuugggccuccauaaaguaggaaacacuacauccccccagccccuccuccccuuccugcacccguacccccaccccuaucacaauuagcauuaaguggucuuugaauaaagucugagugggcggc

SEQ ID NO: 162 - RNA, 142 nt, Artificial Sequence; identical to SEQ ID NO: 104
  source: /note="Description of Artificial Sequence: Synthetic polynucleotide"

SEQ ID NO: 163 - RNA, 142 nt, Artificial Sequence; identical to SEQ ID NO: 105
  source: /note="Description of Artificial Sequence: Synthetic polynucleotide"

SEQ ID NO: 164 - RNA, 142 nt, Artificial Sequence
  source: /note="Description of Artificial Sequence: Synthetic polynucleotide"
ugauaauaggcuggagccucgguggccaugcuucuugccccuugggccuccauaaaguaggaaacacuacauccccccagccccuccuccccuuccugcacccguacccccguggucuuugaauaaagucugagugggcggc

SEQ ID NO: 165 - RNA, 70 nt, Artificial Sequence
  source: /note="Description of Artificial Sequence: Synthetic oligonucleotide"
gggaaauaagaguccauaaaguaggaaacacuacaagaaaagaagaguaagaagaaauauaagagccacc

SEQ ID NO: 166 - RNA, 70 nt, Artificial Sequence
  source: /note="Description of Artificial Sequence: Synthetic oligonucleotide"
gggaaauaagagagaaaagaagaguaauccauaaaguaggaaacacuacagaagaaauauaagagccacc

SEQ ID NO: 167 - RNA, 70 nt, Artificial Sequence
  source: /note="Description of Artificial Sequence: Synthetic oligonucleotide"
gggaaauaagagagaaaagaagaguaagaagaaauauaauccauaaaguaggaaacacuacagagccacc

SEQ ID NO: 168 - RNA, 23 nt, Artificial Sequence
  source: /note="Description of Artificial Sequence: Synthetic oligonucleotide"
accccuaucacaauuagcauuaa

SEQ ID NO: 169 - RNA, 181 nt, Artificial Sequence
  source: /note="Description of Artificial Sequence: Synthetic polynucleotide"
ugauaauagaguagugcuuucuacuuuauggcuggagccucgguggccaugcuucuugccccuugggccaguagugcuuucuacuuuauguccccccagccccucuccccuuccugcacccguacccccaguagugcuuucuacuuuaugguggucuuugaauaaagucugagugggcggc

SEQ ID NO: 170 - RNA, 142 nt, Artificial Sequence; identical to SEQ ID NO: 106
  source: /note="Description of Artificial Sequence: Synthetic polynucleotide"

SEQ ID NO: 171 - RNA, 142 nt, Artificial Sequence; identical to SEQ ID NO: 107
  source: /note="Description of Artificial Sequence: Synthetic polynucleotide"

SEQ ID NO: 172 - RNA, 142 nt, Artificial Sequence; identical to SEQ ID NO: 108
  source: /note="Description of Artificial Sequence: Synthetic polynucleotide"

SEQ ID NO: 173 - RNA, 142 nt, Artificial Sequence; identical to SEQ ID NO: 110
  source: /note="Description of Artificial Sequence: Synthetic polynucleotide"

SEQ ID NO: 174 - RNA, 164 nt, Artificial Sequence; identical to SEQ ID NO: 112
  source: /note="Description of Artificial Sequence: Synthetic polynucleotide"

SEQ ID NO: 175 - RNA, 119 nt, Artificial Sequence
  source: /note="Description of Artificial Sequence: Synthetic polynucleotide"
ugauaauaggcuggagccucgguggccuagcuucuugccccuugggccuccccccagccccuccuccccuuccugcacccguacccccguggucuuugaauaaagucugagugggcggc

SEQ ID NO: 176 - skipped

SEQ ID NO: 177 - RNA, 141 nt, Artificial Sequence
  source: /note="Description of Artificial Sequence: Synthetic polynucleotide"
ugauaauaggcuggagccucgguggccuagcuucuugccccuugggccuccccccagccccuccuccccuuccugcacccguaccccccgcauuauuacucacgguacgaguggucuuugaauaaagucugagugggcggc

SEQ ID NO: 178 - RNA, 188 nt, Artificial Sequence
  source: /note="Description of Artificial Sequence: Synthetic polynucleotide"
ugauaauaguccauaaaguaggaaacacuacagcuggagccucgguggccuagcuucuugccccuugggccuccauaaaguaggaaacacuacauccccccagccccuccuccccuuccugcacccguacccccuccauaaaguaggaaacacuacaguggucuuugaauaaagucugagugggcggc

SEQ ID NO: 179 - RNA, 142 nt, Artificial Sequence
  source: /note="Description of Artificial Sequence: Synthetic polynucleotide"
ugauaauaguccauaaaguaggaaacacuacagcuggagccucgguggccuagcuucuugccccuugggccuccccccagccccuccuccccuuccugcacccguacccccguggucuuugaauaaagucugagugggcggc

SEQ ID NO: 180 - RNA, 142 nt, Artificial Sequence
  source: /note="Description of Artificial Sequence: Synthetic polynucleotide"
ugauaauaggcuggagccucgguggcuccauaaaguaggaaacacuacacuagcuucuugccccuugggccuccccccagccccuccuccccuuccugcacccguacccccguggucuuugaauaaagucugagugggcggc

SEQ ID NO: 181 - RNA, 142 nt, Artificial Sequence
  source: /note="Description of Artificial Sequence: Synthetic polynucleotide"
ugauaauaggcuggagccucgguggccuagcuucuugccccuugggccuccauaaaguaggaaacacuacauccccccagccccuccuccccuuccugcacccguacccccguggucuuugaauaaagucugagugggcggc

SEQ ID NO: 182 - RNA, 142 nt, Artificial Sequence
  source: /note="Description of Artificial Sequence: Synthetic polynucleotide"
ugauaauaggcuggagccucgguggccuagcuucuugccccuugggccuccccccagccccuccuccccuuccugcacccguacccccaccccuaucacaauuagcauuaaguggucuuugaauaaagucugagugggcggc

SEQ ID NO: 183 - RNA, 188 nt, Artificial Sequence
  source: /note="Description of Artificial Sequence: Synthetic polynucleotide"
ugauaauagaccccuaucacaauuagcauuaagcuggagccucgguggccuagcuucuugccccuugggccaccccuaucacaauuagcauuaauccccccagccccuccuccccuuccugcacccguacccccaccccuaucacaauuagcauuaaguggucuuugaauaaagucugagugggcggc

SEQ ID NO: 184 - RNA, 188 nt, Artificial Sequence
  source: /note="Description of Artificial Sequence: Synthetic polynucleotide"
ugauaauagaccccuaucacaauuagcauuaagcuggagccucgguggccuagcuucuugccccuugggccuccauaaaguaggaaacacuacauccccccagccccuccuccccuuccugcacccguacccccaccccuaucacaauuagcauuaaguggucuuugaauaaagucugagugggcggc

SEQ ID NO: 185 - DNA, 18 bp, Artificial Sequence
  source: /note="Description of Artificial Sequence: Synthetic oligonucleotide"
attgggcacccgtaaggg

SEQ ID NO: 186 - protein, 25 aa, Artificial Sequence
  source: /note="Description of Artificial Sequence: Synthetic peptide"
GSGVKQTLNFDLLKLAGDVESNPGP

SEQ ID NO: 187 - protein, 21 aa, Artificial Sequence
  source: /note="Description of Artificial Sequence: Synthetic peptide"
GSGEGRGSLLTCGDVEENPGP

SEQ ID NO: 188 - protein, 22 aa, Artificial Sequence
  source: /note="Description of Artificial Sequence: Synthetic peptide"
GSGATNFSLLKQAGDVEENPGP

SEQ ID NO: 189 - protein, 23 aa, Artificial Sequence
  source: /note="Description of Artificial Sequence: Synthetic peptide"
GSGQCTNYALLKLAGDVESNPGP

SEQ ID NO: 190 - protein, 20 aa, Artificial Sequence
  source: /note="Description of Artificial Sequence: Synthetic peptide"
  SITE (1)..(20): /note="This sequence may encompass 2-5 'Gly Gly Gly Ser' repeating units"
GGGSGGGSGGGSGGGSGGGS

SEQ ID NO: 191 - RNA, 66 nt, Artificial Sequence
  source: /note="Description of Artificial Sequence: Synthetic oligonucleotide"
ggaagcggagcuacuaacuucagccugcugaagcaggcuggagacguggaggagaacccuggaccu

SEQ ID NO: 192 - DNA, 108 bp, Artificial Sequence
  source: /note="Description of Artificial Sequence: Synthetic oligonucleotide"
  source: /note="Description of Combined DNA/RNA Molecule: Synthetic oligonucleotide"
uccggacucagauccggggaucucaaaauugucgcuccugucaaacaaacucuuaacuuugauuuacucaaacuggctggggauguagaaagcaauccaggtccacuc

SEQ ID NO: 193 - RNA, 92 nt, Artificial Sequence; identical to SEQ ID NO: 88
  source: /note="Description of Artificial Sequence: Synthetic oligonucleotide"

SEQ ID NO: 194 - protein, 357 aa, Artificial Sequence
  source: /note="Description of Artificial Sequence: Synthetic polypeptide"
MEEGMNVLHDFGIQSTHYLQVNYQDSQDWFILVSVIADLRNAFYVLFPIWFHLQEAVGIKLLWVAVIGDWLNLVFKWILFGQRPYWWVLDTDYYSNTSVPLIKQFPVTCETGPGSPSGHAMGTAGVYYVMVTSTLSIFQGKIKPTYRFRCLNVILWLGFWAVQLNVCLSRIYLAAHFPHQVVAGVLSGIAVAETFSHIHSIYNASLKKYFLITFFLFSFAIGFYLLLKGLGVDLLWTLEKAQRWCEQPEWVHIDTTPFASLLKNLGTLFGLGLALNSSMYRESCKGKLSKWLPFRLSCIVASLVLLHVFDSLKPPSQVELVFYVLSFCKSAVVPLASVSVIPYCLAQVLGQPHKKSL

SEQ ID NO: 195 - protein, 357 aa, Artificial Sequence
  source: /note="Description of Artificial Sequence: Synthetic polypeptide"
MEEGMNVLHDFGIQSTHYLQVNYQDSQDWFILVSVIADLRNAFYVLFPIWFHLQEAVGIKLLWVAVIGDWLNLVFKWILFGQRPYWWVLDTDYYSNTSVPLIKQFPVTCETGPGSPSGHAMGTAGVYYVMVTSTLSIFRGKIKPTYRFRCLNVILWLGFWAVQLNVCLSRIYLAAHFPHQVVAGVLSGIAVAETFSHIHSIYNASLKKYFLITFFLFSFAIGFYLLLKGLGVDLLWTLEKAQRWCEQPEWVHIDTTPFASLLKNLGTLFGLGLALNSSMYRESCKGKLSKWLPFRLSSIVASLVLLHVFDSLKPPSQVELVFYVLSFCKSAVVPLASVSVIPYCLAQVLGQPHKKSL

SEQ ID NO: 196 - protein, 357 aa, Artificial Sequence
  source: /note="Description of Artificial Sequence: Synthetic polypeptide"
MEEGMNVLHDFGIQSTHYLQVNYQDSQDWFILVSVIADLRNAFYVLFPIWFHLQEAVGIKLLWVAVIGDWLNLVFKWILFGQRPYWWVLDTDYYSNTSVPLIKQFPVTCETGPGSPSGHAMGTAGVYYVMVTSTLSIFQGKIKPTYRFRCLNVILWLGFWAVQLNVCLSRIYLAAHFPHQVVAGVLSGIAVAETFSHIHSIYNASLKKYFLITFFLFSFAIGFYLLLKGLGVDLLWTLEKAQRWCERPEWVHIDTTPFASLLKNLGTLFGLGLALNSSMYRESCKGKLSKWLPFRLSSIVASLVLLHVFDSLKPPSQVELVFYVLSFCKSAVVPLASVSVIPYCLAQVLGQPHKKSL

SEQ ID NO: 197 - protein, 357 aa, Artificial Sequence
  source: /note="Description of Artificial Sequence: Synthetic polypeptide"
MEEGMNVLHDFGIQSTHYLQVNYQDSQDWFILVSVIADLRNAFYVLFPIWFHLQEAVGIKLLWVAVIGDWLNLVFKWILFGQRPYWWVLDTDYYSNTSVPLIKQFPVTCETGPGSPSGHAMGTAGVYYVMVTSTLSIFQGKKKPTYRFRCLNVILWLGFWAVQLNVCLSRIYLAAHFPHQVVAGVLSGIAVAETFSHIHSIYNASLKKYFLITFFLFSFAIGFYLLLKGLGVDLLWTLEKAQRWCEQPEWVHIDTTPFASLLKNLGTLFGLGLALNSSMYRESCKGKLSKWLPFRLSSIVASLVLLHVFDSLKPPSQVELVFYVLSFCKSAVVPLASVSVIPYCLAQVLGQPHKKSL

SEQ ID NO: 198 - protein, 357 aa, Artificial Sequence
  source: /note="Description of Artificial Sequence: Synthetic polypeptide"
MEEGMNVLHDFGIQSTHYLQVNYQDSQDWFILVSVIADLRNAFYVLFPIWFHLQEAVGIKLLWVAVIGDWLNLVFKWILFGQRPYWWVLDTDYYSNTSVPLIKQFPVTCETGPGSPSGHAMGTAGVYYVMVTSTLSIFQGKIKPTYRFRCLNVILWLGFWAVQLNVCLSRIYLAAHFPHQVVAGVLSGIAVAETFSHIHSIYNASLKKYFLITFFLFSFAIGFYLLLKGLGVDLLWTLEKAQRWCEQPEWVHIDTTPFASLLKNLGTLFGLGLALNSSMYRESCKGKLSKWLPFRLGSIVASLVLLHVFDSLKPPSQVELVFYVLSFCKSAVVPLASVSVIPYCLAQVLGQPHKKSL

SEQ ID NO: 199 - protein, 357 aa, Homo sapiens
MEEGMNVLHDFGIQSTHYLQVNYQDSQDWFILVSVIADLRNAFYVLFPIWFHLQEAVGIKLLWVAVIGDWLNLVFKWILFGQRPYWWVLDTDYYSNTSVPLIKQFPVTCETGPGSPSGHAMGTAGVYYVMVTSTLSIFQGKIKPTYRFRCLNVILWLGFWAVQLNVCLSRIYLAAHFPHQVVAGVLSGIAVAETFSHIHSIYNASLKKYFLITFFLFSFAIGFYLLLKGLGVDLLWTLEKAQRWCEQPEWVHIDTTPFASLLKNLGTLFGLGLALNSSMYRESCKGKLSKWLPFRLSSIVASLVLLHVFDSLKPPSQVELVFYVLSFCKSAVVPLASVSVIPYCLAQVLGQPHKKSL

SEQ ID NO: 200 - protein, 357 aa, Artificial Sequence
  source: /note="Description of Artificial Sequence: Synthetic polypeptide"
MEEGMNVLHDFGIQSTHYLQVNYQDSQDWFILVSVIADLRNAFYVLFPIWFHLQEAVGIKLLWVAVIGDWLNLVFKWILFGQRPYWWVLDTDYYSNTSVPLIKQFPVTCETGPGSPSGHAMGTAGVYYVMVTSTLSIFQGKIKPTYRFRCLNVILWLGFWAVQLNVCLSRIYLAAHFPHQVVAGVLSGIAVAETFSHIHSIYNASLKKYFLITFFLFSFAIGFYLLLKGLGVDLLWTLEKAQRWCEQPEWVHIDTTPFASLLKNLGTLFGLGLALNSSMYRESCKGKLSKWLPFRLSSIVASLVLLHLFDSLKPPSQVELVFYVLSFCKSAVVPLASVSVIPYCLAQVLGQPHKKSL

SEQ ID NO: 201 - protein, 357 aa, Artificial Sequence
  source: /note="Description of Artificial Sequence: Synthetic polypeptide"
MEEGMNVLHDFGIQSTHYLQVNYQDSQDWFILVSVIADLRNAFYVLFPIWFHLQEAVGIKLLWVAVIGDWLNLVFKWILFGQRPYWWVLDTDYYSNTSVPLIKQFPVTCETGPGSPSGHAMGTAGVYYVMVTSTLSIFQGKIKPTYRFRCLNVILWLGFWAVQLNVCLSRIYLAAHFPHQVVAGVLSGIAVAETFSHIHSIYNASLKKYFLITFFLFSFAIGFYLLLKGLGVDLLWTLEKAQRWCEQPEWVHIDTTPFASLLKNLGTLFGLGLALNSSMYRESCKGKLSKWLPFRLSSIVASLVLLHVFDSLKPPSQVELIFYVLSFCKSAVVPLASVSVIPYCLAQVLGQPHKKSL

SEQ ID NO: 202 - protein, 357 aa, Artificial Sequence
  source: /note="Description of Artificial Sequence: Synthetic polypeptide"
MEEGMNVLHDFGIQSTHYLQVNYQDSQDWFILVSVIADLRNAFYVLFPIWFHLQEAVGIKLLWVAVIGDWLNLVFKWILFGQRPYWWVLDTDYYSNTSVPLIKQFPVTCETGPGSPSGHAMGTAGVYYVMVTSTLSIFQGKIKPTYRFRCLNVILWLGFWAVQLNVCLSRIYLAAHFPHQVVAGVLSGIAVAETFSHIHSIYNASLKKYFLITFFLFSFAIGFYLLLKGLGVDLLWTLEKAQRWCEQPEWVHIDTTPFASLLKNLGTLFGLGLALNSSMYRESCKGKLSKWLPFRLSSIVASLVLLHVFDSLKPPSQVELLFYVLSFCKSAVVPLASVSVIPYCLAQVLGQPHKKSL

SEQ ID NO: 203 - protein, 357 aa, Artificial Sequence
  source: /note="Description of Artificial Sequence: Synthetic polypeptide"
MEEGMNVLHDFGIQSTHYLQVNYQDSQDWFILVSVIADLRNAFYVLFPIWFHLQEAVGIKLLWVAVIGDWLNLVFKWILFGQRPYWWVLDTDYYSNTSVPLIKQFPVTCETGPGSPSGHAMGTAGVYYVMVTSTLSIFQGKIKPTYRFRCLNVILWLGFWAVQLNVCLSRIYLAAHFPHQVVAGVLSGIAVAETFSHIHSIYNASLKKYFLITFFLFSFAIGFYLLLKGLGVDLLWTLEKAQRWCEQPEWVHIDTTPFASLLKNLGTLFGLGLALNSSMYRESCKGKLSKWLPFRLSSIVASLVLLHVFDSLKPPSQVELVFYVLSFCKSAVVPLASVSLIPYCLAQVLGQPHKKSL

SEQ ID NO: 204 - protein, 357 aa, Artificial Sequence
  source: /note="Description of Artificial Sequence: Synthetic polypeptide"
MEEGMNVLHDFGIQSTHYLQVNYQDSQDWFILVSVIADLRNAFYVLFPIWFHLQEAVGIKLLWVAVIGDWLNLVFKWILFGQRPYWWVLDTDYYSNTSVPLIKQFPVTCETGPGSPSGHAMGTAGVYYVMVTSTLSIFQGKIKPTYRFRCLNVILWLGFWAVQLNVCLSRIYLAAHFPHQVVAGVLSGIAVAETFSHIHSIYNASLKKYFLITFFLFSFAIGFYLLLKGLGVDLLWTLEKAQRWCEQPEWVHIDTTPFASLLKNLGTLFGLGLALNSSMYRESCKGKLSKWLPFRLSSIVASLVLLHVFDSLKPPSQVELVFYVLSFCKSAAVPLASVSVIPYCLAQVLGQPHKKSL

SEQ ID NO: 205 - protein, 357 aa, Artificial Sequence
  source: /note="Description of Artificial Sequence: Synthetic polypeptide"
MEEGMNVLHDFGIQSTHYLQVNYQDSQDWFILVSVIADLRNAFYVLFPIWFHLQEAVGIKLLWVAVIGDWLNLVFKWILFGQRPYWWVLDTDYYSNTSVPLIKQFPVTCETGPGSPSGHAMGTAGVYYVMVTSTLSIFRGKIKPTYRFRCLNVILWLGFWAVQLNVCLSRIYLAAHFPHQVVAGVLSGIAVAETFSHIHSIYNASLKKYFLITFFLFSFAIGFYLLLKGLGVDLLWTLEKAQRWCERPEWVHIDTTPFASLLKNLGTLFGLGLALNSSMYRESCKGKLSKWLPFRLSCIVASLVLLHVFDSLKPPSQVELVFYVLSFCKSAVVPLASVSVIPYCLAQVLGQPHKKSL

SEQ ID NO: 206 - protein, 357 aa, Artificial Sequence
  source: /note="Description of Artificial Sequence: Synthetic polypeptide"
MEEGMNVLHDFGIQSTHYLQVNYQDSQDWFILVSVIADLRNAFYVLFPIWFHLQEAVGIKLLWVAVIGDWLNLVFKWILFGQRPYWWVLDTDYYSNTSVPLIKQFPVTCETGPGSPSGHAMGTAGVYYVMVTSTLSIFQGKIKPTYRFRCLNVILWLGFWAVQLNVCLSRIYLAAHFPHQVVAGVLSGIAVAETFSHIHSIYNASLKKYFLITFFLFSFAIGFYLLLKGLGVDLLWTLEKAQRWCERPEWVHIDTTPFASLLKNLGTLFGLGLALNSSMYRESCKGKLSKWLPFRLSCIVASLVLLHVFDSLKPPSQVELVFYVLSFCKSAVVPLASVSVIPYCLAQVLGQPHKKSL

SEQ ID NO: 207 - RNA, 1071 nt, Artificial Sequence
  source: /note="Description of Artificial Sequence: Synthetic polynucleotide"
auggaggaaggaaugaauguucuccaugacuuugggauccagucaacacauuaccuccaggugaauuaccaagacucccaggacugguucaucuugguguccgugaucgcagaccucaggaaugccuucuacguccucuuccccaucugguuccaucuucaggaagcugugggcauuaaacuccuuuggguagcugugauuggagacuggcucaaccucgucuuuaaguggauucucuuuggacagcguccauacugguggguuuuggauacugacuacuacagcaacacuuccgugccccugauaaagcaguucccuguaaccugugagacuggaccagggagccccucuggccaugccaugggcacagcagguguauacuacgugauggucacaucuacucuuuccaucuuucagggaaagauaaagccgaccuacagauuucggugcuugaaugucauuuugugguugggauucugggcugugcagcugaaugucugucugucacgaaucuaccuugcugcucauuuuccucaucaaguuguugcuggaguccugucaggcauugcuguugcagaaacuuucagccacauccacagcaucuauaaugccagccucaagaaauauuuucucauuaccuucuuccuguucagcuucgccaucggauuuuaucugcugcucaagggacuggguguagaccuccuguggacucuggagaaagcccagagguggugcgagaggccagaauggguccacauugacaccacacccuuugccagccuccucaagaaccugggcacgcucuuuggccuggggcuggcucucaacuccagcauguacagggagagcugcaaggggaaacucagcaaguggcucccauuccgccucagcuguauuguagccucccucguccuccugcacgucuuugacuccuugaaacccccaucccaagucgagcuggucuucuacgucuuguccuucugcaagagugcgguagugccccuggcauccgucagugucauccccuacugccucgcccagguccugggccagccgcacaagaagucguug

SEQ ID NO: 208 - protein, 357 aa, Artificial Sequence
  source: /note="Description of Artificial Sequence: Synthetic polypeptide"
MEEGMNVLHDFGIQSTHYLQVNYQDSQDWFILVSVIADLRNAFYVLFPIWFHLQEAVGIKLLWVAVIGDWLNLVFKWILFGQRPYWWVLDTDYYSNTSVPLIKQFPVTCETGPGSPSGHAMGTAGVYYVMVTSTLSIFQGKIKPTYRFRCLNVILWLGFWAVQLNVCLSRIYLAAHFPHQVVAGVLSGIAVAETFSHIHSIYNASLKKYFLITFFLFSFAIGFYLLLKGLGVDLLWTLEKAQRWCEQPEWVHIDTTPFASLLKNLGTLFGLGLALNSSMYRESCKGKLSKWLPFRLSAIVASLVLLHVFDSLKPPSQVELVFYVLSFCKSAVVPLASVSVIPYCLAQVLGQPHKKSL

SEQ ID NO: 209 - protein, 357 aa, Artificial Sequence
  source: /note="Description of Artificial Sequence: Synthetic polypeptide"
MEEGMNVLHDFGIQSTHYLQVNYQDSQDWFILVSVIADLRNAFYVLFPIWFHLQEAVGIKLLWVAVIGDWLNLVFKWILFGQRPYWWVLDTDYYSNTSVPLIKQFPVTCETGPGSPSGHAMGTAGVYYVMVTSTLSIFRGKKKPTYRFRCLNVILWLGFWAVQLNVCLSRIYLAAHFPHQVVAGVLSGIAVAETFSHIHSIYNASLKKYFLITFFLFSFAIGFYLLLKGLGVDLLWTLEKAQRWCERPEWVHIDTTPFASLLKNLGTLFGLGLALNSSMYRESCKGKLSKWLPFRLGCIVASLVLLHLFDSLKPPSQVELIFYVLSFCKSAVVPLASVSLIPYCLAQVLGQPHKKSL

SEQ ID NO: 210 - RNA, 47 nt, Artificial Sequence
  source: /note="Description of Artificial Sequence: Synthetic oligonucleotide"
aggaaauaagagagaaaagaagaguaagaagaaauauaagagccacc

SEQ ID NO: 211 - RNA, 57 nt, Artificial Sequence
  source: /note="Description of Artificial Sequence: Synthetic oligonucleotide"
aggaaauaagagagaaaagaagaguaagaagaaauauaagaccccggcgccgccacc

SEQ ID NO: 212 - RNA, 141 nt, Artificial Sequence
  source: /note="Description of Artificial Sequence: Synthetic polynucleotide"
ugauaauaggcuggagccucgguggccaugcuucuugccccuugggccuccccccagccccuccuccccuuccugcacccguaccccccaaacaccauugucacacuccaguggucuuugaauaaagucugagugggcggc

SEQ ID NO: 213 - RNA, 141 nt, Artificial Sequence
  source: /note="Description of Artificial Sequence: Synthetic polynucleotide"
ugauaauaggcuggagccucgguggccuagcuucuugccccuugggccuccccccagccccuccuccccuuccugcacccguaccccccaaacaccauugucacacuccaguggucuuugaauaaagucugagugggcggc

SEQ ID NO: 214 - RNA, 1237 nt, Artificial Sequence
  source: /note="Description of Artificial Sequence: Synthetic polynucleotide"
aggaaauaagagagaaaagaagaguaagaagaaauauaagagccaccauggaggagggcaugaacgugcuucacgacuucggcauccagucaacccauuaccuacaggugaacuaucaggacucccaggauugguucauccucgugagcgugaucgccgaucuaagaaacgcauucuacguguuguucccaaucugguuccaccugcaggaagcugugggcaucaagcuccuuuggguggccgugauuggcgauuggcugaaccugguguucaaguggauucucuucggucagcggccuuacugguggguguuggauaccgacuauuacaguaacaccucuguuccgcugaucaagcaguucccugucaccugcgaaaccggaccuggcuccccuuccggccacgccaugggcaccgccggcguguacuacgugauggugacauccacccugagcaucuuccagggcaagaucaagccuaccuacagauucaggugccugaacguuaucuuguggcugggauucugggcagugcagcucaacgugugccugagcaggaucuaucucgcagcccacuucccacaucaggucguggccggcguacugagcggaaucgccguggcugaaaccuucagccauauccacagcaucuacaaugccucccugaagaaguacuuccuuauuacauucuuccuguucucuuucgccaucggcuucuaucugcugcuaaagggccugggcgucgaccuccuguggacccuggagaaggcccagagauggugcgaacaaccugagugggugcacaucgacaccacuccguucgcuagccugcucaagaaccugggcacucuuuucggccugggccuggcccucaauagcagcauguaccgggagagcuguaagggaaagcuguccaaguggcucccuuucagacuuagcugcaucguggcgucucucgugcugcugcacguguucgacagccugaagccuccuucgcagguggagcugguguucuacgugcugagcuucugcaagagcgcgguggugccacuggcaagugucagcgugaucccuuauugccuggcccaggugcugggccagccucauaagaagucccugugauaauaggcuggagccucgguggccuagcuucuugccccuugggccuccccccagccccuccuccccuuccugcacccguacccccguggucuuugaauaaagucugagugggcggc

SEQ ID NO: 215 - RNA, 1306 nt, Artificial Sequence
  source: /note="Description of Artificial Sequence: Synthetic polynucleotide"
aggaaauaagagagaaaagaagaguaagaagaaauauaagagccaccauggaggagggcaugaacgugcuucacgacuucggcauccagucaacccauuaccuacaggugaacuaucaggacucccaggauugguucauccucgugagcgugaucgccgaucuaagaaacgcauucuacguguuguucccaaucugguuccaccugcaggaagcugugggcaucaagcuccuuuggguggccgugauuggcgauuggcugaaccugguguucaaguggauucucuucggucagcggccuuacugguggguguuggauaccgacuauuacaguaacaccucuguuccgcugaucaagcaguucccugucaccugcgaaaccggaccuggcuccccuuccggccacgccaugggcaccgccggcguguacuacgugauggugacauccacccugagcaucuuccagggcaagaucaagccuaccuacagauucaggugccugaacguuaucuuguggcugggauucugggcagugcagcucaacgugugccugagcaggaucuaucucgcagcccacuucccacaucaggucguggccggcguacugagcggaaucgccguggcugaaaccuucagccauauccacagcaucuacaaugccucccugaagaaguacuuccuuauuacauucuuccuguucucuuucgccaucggcuucuaucugcugcuaaagggccugggcgucgaccuccuguggacccuggagaaggcccagagauggugcgaacaaccugagugggugcacaucgacaccacuccguucgcuagccugcucaagaaccugggcacucuuuucggccugggccuggcccucaauagcagcauguaccgggagagcuguaagggaaagcuguccaaguggcucccuuucagacuuagcugcaucguggcgucucucgugcugcugcacguguucgacagccugaagccuccuucgcagguggagcugguguucuacgugcugagcuucugcaagagcgcgguggugccacuggcaagugucagcgugaucccuuauugccuggcccaggugcugggccagccucauaagaagucccugugauaauaguccauaaaguaggaaacacuacagcuggagccucgguggccuagcuucuugccccuugggccuccauaaaguaggaaacacuacauccccccagccccuccuccccuuccugcacccguacccccuccauaaaguaggaaacacuacaguggucuuugaauaaagucugagugggcggc

SEQ ID NO: 216 - protein, 4 aa, Artificial Sequence
  source: /note="Description of Artificial Sequence: Synthetic peptide"
GGGS

SEQ ID NO: 217 - RNA, 1306 nt, Artificial Sequence
  source: /note="Description of Artificial Sequence: Synthetic polynucleotide"
gggaaauaagagagaaaagaagaguaagaagaaauauaagagccaccauggaggagggcaugaacgugcuucacgacuucggcauccagucaacccauuaccuacaggugaacuaucaggacucccaggauugguucauccucgugagcgugaucgccgaucuaagaaacgcauucuacguguuguucccaaucugguuccaccugcaggaagcugugggcaucaagcuccuuuggguggccgugauuggcgauuggcugaaccugguguucaaguggauucucuucggucagcggccuuacugguggguguuggauaccgacuauuacaguaacaccucuguuccgcugaucaagcaguucccugucaccugcgaaaccggaccuggcuccccuuccggccacgccaugggcaccgccggcguguacuacgugauggugacauccacccugagcaucuuccagggcaagaucaagccuaccuacagauucaggugccugaacguuaucuuguggcugggauucugggcagugcagcucaacgugugccugagcaggaucuaucucgcagcccacuucccacaucaggucguggccggcguacugagcggaaucgccguggcugaaaccuucagccauauccacagcaucuacaaugccucccugaagaaguacuuccuuauuacauucuuccuguucucuuucgccaucggcuucuaucugcugcuaaagggccugggcgucgaccuccuguggacccuggagaaggcccagagauggugcgaacaaccugagugggugcacaucgacaccacuccguucgcuagccugcucaagaaccugggcacucuuuucggccugggccuggcccucaauagcagcauguaccgggagagcuguaagggaaagcuguccaaguggcucccuuucagacuuagcugcaucguggcgucucucgugcugcugcacguguucgacagccugaagccuccuucgcagguggagcugguguucuacgugcugagcuucugcaagagcgcgguggugccacuggcaagugucagcgugaucccuuauugccuggcccaggugcugggccagccucauaagaagucccugugauaauaguccauaaaguaggaaacacuacagcuggagccucgguggccuagcuucuugccccuugggccuccauaaaguaggaaacacuacauccccccagccccuccuccccuuccugcacccguacccccuccauaaaguaggaaacacuacaguggucuuugaauaaagucugagugggcggc

SEQ ID NO: 218 - RNA, 150 nt, Artificial Sequence
  source: /note="Description of Artificial Sequence: Synthetic polynucleotide"
  misc_feature (1)..(150): /note="This sequence may encompass 75-150 nucleotides"
aaaaaaaaaaaaaaaaaaaaaaaaaaaaaaaaaaaaaaaaaaaaaaaaaaaaaaaaaaaaaaaaaaaaaaaaaaaaaaaaaaaaaaaaaaaaaaaaaaaaaaaaaaaaaaaaaaaaaaaaaaaaaaaaaaaaaaaaaaaaaaaaaaaaaa

SEQ ID NO: 219 - RNA, 150 nt, Artificial Sequence; identical to SEQ ID NO: 218
  source: /note="Description of Artificial Sequence: Synthetic polynucleotide"
  misc_feature (1)..(150): /note="This sequence may encompass 85-150 nucleotides"

SEQ ID NO: 220 - RNA, 150 nt, Artificial Sequence; identical to SEQ ID NO: 218
  source: /note="Description of Artificial Sequence: Synthetic polynucleotide"
  misc_feature (1)..(150): /note="This sequence may encompass 90-150 nucleotides"

SEQ ID NO: 221 - RNA, 120 nt, Artificial Sequence
  source: /note="Description of Artificial Sequence: Synthetic polynucleotide"
  misc_feature (1)..(120): /note="This sequence may encompass 90-120 nucleotides"
aaaaaaaaaaaaaaaaaaaaaaaaaaaaaaaaaaaaaaaaaaaaaaaaaaaaaaaaaaaaaaaaaaaaaaaaaaaaaaaaaaaaaaaaaaaaaaaaaaaaaaaaaaaaaaaaaaaaaaaa

SEQ ID NO: 222 - RNA, 130 nt, Artificial Sequence
  source: /note="Description of Artificial Sequence: Synthetic polynucleotide"
  misc_feature (1)..(130): /note="This sequence may encompass 90-130 nucleotides"
aaaaaaaaaaaaaaaaaaaaaaaaaaaaaaaaaaaaaaaaaaaaaaaaaaaaaaaaaaaaaaaaaaaaaaaaaaaaaaaaaaaaaaaaaaaaaaaaaaaaaaaaaaaaaaaaaaaaaaaaaaaaaaaaaa

SEQ ID NO: 223 - RNA, 100 nt, Artificial Sequence
  source: /note="Description of Artificial Sequence: Synthetic polynucleotide"
aaaaaaaaaaaaaaaaaaaaaaaaaaaaaaaaaaaaaaaaaaaaaaaaaaaaaaaaaaaaaaaaaaaaaaaaaaaaaaaaaaaaaaaaaaaaaaaaaaaa

SEQ ID NO: 224 - protein, 4 aa, Unknown
  source: /note="Description of Unknown: 2A cleavable peptide"
NPGP

SEQ ID NO: 225 - RNA, 30 nt, Artificial Sequence
  source: /note="Description of Artificial Sequence: Synthetic oligonucleotide"
  misc_feature (1)..(30): /note="This sequence may encompass 1-10 'ccg' repeating units"
ccgccgccgccgccgccgccgccgccgccg

SEQ ID NO: 226 - RNA, 24 nt, Artificial Sequence
  source: /note="Description of Artificial Sequence: Synthetic oligonucleotide"
  misc_feature (1)..(24): /note="This sequence may encompass 2-8 'ccg' repeating units"
ccgccgccgccgccgccgccgccg

SEQ ID NO: 227 - RNA, 18 nt, Artificial Sequence
  source: /note="Description of Artificial Sequence: Synthetic oligonucleotide"
  misc_feature (1)..(18): /note="This sequence may encompass 3-6 'ccg' repeating units"
ccgccgccgccgccgccg

SEQ ID NO: 228 - RNA, 15 nt, Artificial Sequence
  source: /note="Description of Artificial Sequence: Synthetic oligonucleotide"
  misc_feature (1)..(15): /note="This sequence may encompass 4-5 'ccg' repeating units"
ccgccgccgccgccg

SEQ ID NO: 229 - RNA, 15 nt, Artificial Sequence
  source: /note="Description of Artificial Sequence: Synthetic oligonucleotide"
  misc_feature (1)..(15): /note="This sequence may encompass 1-5 'ccg' repeating units"
ccgccgccgccgccg

SEQ ID NO: 230 - RNA, 12 nt, Artificial Sequence
  source: /note="Description of Artificial Sequence: Synthetic oligonucleotide"
ccgccgccgccg

SEQ ID NO: 231 - RNA, 15 nt, Artificial Sequence
  source: /note="Description of Artificial Sequence: Synthetic oligonucleotide"
ccgccgccgccgccg

SEQ ID NO: 232 - RNA, 30 nt, Artificial Sequence
  source: /note="Description of Artificial Sequence: Synthetic oligonucleotide"
  misc_feature (1)..(30): /note="This sequence may encompass 1-10 'gcc' repeating units"
gccgccgccgccgccgccgccgccgccgcc

SEQ ID NO: 233 - RNA, 120 nt, Artificial Sequence; identical to SEQ ID NO: 221
  source: /note="Description of Artificial Sequence: Synthetic polynucleotide"

SEQ ID NO: 234 - DNA, 120 bp, Artificial Sequence
  source: /note="Description of Artificial Sequence: Synthetic polynucleotide"
tttttttttttttttttttttttttttttttttttttttttttttttttttttttttttttttttttttttttttttttttttttttttttttttttttttttttttttttttttttttt

SEQ ID NO: 235 - RNA, 150 nt, Artificial Sequence; identical to SEQ ID NO: 218
  source: /note="Description of Artificial Sequence: Synthetic polynucleotide"
  misc_feature (1)..(150): /note="This sequence may encompass 50-150 nucleotides"